European Patent Specification EP 3 320 100 B1, published August 28, 2024. Title: Fowl Adenovirus 9 (FADV-9) vector system and associated methods. Applicant: University of Guelph. The sequence listing filed with the application follows.

SEQUENCE LISTING (68 sequences)

SEQ ID NO: 1 - DNA, 45063 bp, Fowl aviadenovirus D
  whole genome (1)..(45063)
catcatctatatatacctacatgaatgacgctgctgtcacctcgcactaccgctcccgcccgctagatggcaaaattgctccaccaaagtatttccgtgatacaaagtccggactgggcgcggcgaatacgtgccgggcgaggcacggagccgactttctggcaccgatagcaataaatgggcgttcccttgcgtgcggaattgcgccggcacagtcccaatggcttgggagcggtccagaaagcgattagtttttgcgtacgcacgcgaaagctatttttgcagcacttacttccttatttgtttacaaccgcctccgcctgtgtgtaatttaaaatttgtacataccgttccgatcgccgtacttgggcttggaacgcggacttcgagtccctaaattgatttatggtgtcttaatcagcgctttttgtgccacgttgtgcgttctccgttgacctttgaaaaggcgcgtggtatttctcggtgtgtttttcgggcggattacgcgttacgtgatcgttttatggcgggctccgggcgtataacagtggagcggctgatcgtcagagcacggatgagcgagcagccggactcaccgccggagctctatccgtctctcctggtcctgcgggtgaacccggttccccgtactccgttcgttttggacatcagccgtttgcccgtggtgccggagcgcattttgctgcacgactttccgaacggaccctggtcggaaacgatttggtacgggaagatcactcagcgggagctgaaccaggcgctagagtctatcgtggacgtgctttaggtaatttcctccgttctttttcccgtttaggtgaggagatgtctttcgattccggttgccccccgactccaccggtaaagctgctgttcaagaagcattccccgtttgccgtgacgccccagcgtgctacctcgggggctgccggttacgacttgtgcagctcggcggacgtggtggtgccgccgaagagccggtctctcattccgaccgacctttcttttcaattcccccgaggcgtgtacgggcgcatagcccctcgttcgggcttggccgtaaagttttttatcgatgtgggagccggtgttatcgatagcgattaccggggcatcgttagcgtcctccttttcaatttttcggaccacaatttcaacgtccgtcggggcgatcgcatagctcagttaattttggagcgtcatttgacgcccgacttggaagagcgatcgggcttagacgagacggccaggggtgcagccggtttcggctccaccggcggttttgatacaggggtctgtccctcctccttttcttaggaattgaccgagagcgaggcggcggacgaagtggatttcgccgttcaactggcggccgctctcgaggcagataacgaggctactgcgggttgcttctgcgaagccgactccgggaaaaacacctgttctctgtgttcttggaactgtatcattctttaggtatgattgtttctgtttggaccctcgttgtagagctcgttaacgcgtgggatcgtttgtgtggtcgtcgggcttaccgctattacgcggatcgcgagctgttgtggcaagtgcacgagagtctgcggtccgccttggagaagacggtcggtgtcggaagaggcttggcccgcatcggcgacggtgaaaacgggtatttcggaggaggcggcgaagctgttcgcgacaattgacgacatgtcgatcgaagattggttcctcgttttcgtagtgcttttcgctattctgtcttttatgtgggggatgttcttggggatgctttgcgggccaggcgatttggatttcgcgggttactgggactggtatttccgtgtttgtaacgcgagggttccttaataaatgtcttttcgtaacgttaattccgcgtttgggttttgctttttgcagacgggatgtcgggctcgagggatcgctattggtccttggtcgaatctctgataaatagagggatcgtgacccgtcagcagtggtatttcaacgaccgctccgagtacgggtattacacgaagcgctacagaggcgcgatgaaattgtccaacttgttccgcgacgtgcgtcgtcacatgttctggacaaaatgtttggccgactacatgttgacccccgaaaccgactttcttcaaatcgaggagaatccgttttattcggtgttttcgaaaaacggctacgatcccgctctcgtgggctcgatgttgctggcttgggccgcgcggcagtcgaagcgcaataccgtttggattaggggagcgcccgtgacgggagctccttacttggcggaagcgatcgcttactgctgcccgttgatgacgtgcgtcgattggcgcaacaagcagaatccttttgagaaggggttcgagtctttgctgttttggtgggacggcgggcacgtgccgcaccgctgcgtggccttgtgtcgccaggtgtttaggggcgaaaacgtcatgtttccccgggaagacggtcaaatgagcgaattggtgcgtacgcccgtgttgttgtactctgaacacgacgcttgtcgcacgttagtcaagtggggcgtgttcagtgatgagttttctgacggtttacgtaattccatgtattgtttagacttgtccgcgcccatggaaggcgctcagtgcgtcacttgtgccgacgctcgcgcgttttttacgtgggcttacccgcgacgcatggattttgactgtttttgagcgcgtgtgacgcgtgtttcgagtttaccaataaagactcagaacgcattttccgtgtgaccgatgctttttattgttaaatttcaacgggaaagcttgcaaaacggatagcatatgacgactagcctaaaggggaaggtttcgaggttgtcctggacgcgacgacaacagcgcattaagctgttgttaccgtaggagggagtgatgaatatctcgtaaccgcctcgtatgcgggataaggcgtaattattgcggacggcgcggtgggtcagcaagtcgtgcagaggggccagagggttcaggatgtagtcgagtcgtcccgtatcgtcgtcgggggcggtggagatgagtaagaggttgaaattggtgatgttaacgagaggataggggttgttcgcgcgctcttcttcaaagtactcgtacactttatccaaccagtatgtgcacacgactttgctcgctgcttgacacatgaggctgtagggattggtgcaggtgcaatcgtatcggatttgaggcaagggggattgctgctcgaggtcttcggtaacggaccagaatttattgtacagacgacagcgcgccctgcatttgggcatgctgtattcgggcagtatttcttcgaaggtgacggtgtccttcctggggaacggaaacatgcgttctccgtgaagaaactctaagaaaaagatgtcaagagcgaggtgagcgggtgcttccagctgggcttctttgcattctagcgtgagagagtgcacgctgtcctgcggaaagagagaaaattacaggaacacggtgatgacggggtacgggaacttttgcatgagtctcaggaagcacggtatgagtgtgtaatccctgtgcgaccgcggtaacgcgatgcgaatgtgtccgtcgaccacttctatcttggcgaagggtttggaggaatacacgaataggttgatgacgccgtcgatgatttcgatgggaggtctgccgtgacatcggaagcagtgcgtgcaacgttttcggacgtattggtcgaaatggatgggaaacgggttttccgcgatggggtacgcggtgagtttggcgtgccactccatggtgagtgtggcggctagggactgacaaaagagcgagagcggctcctcgcactcgcatacgtagctcgcgacccattctcccatccatttccgacctccgtcctctacgtcggctaataggttgctaattttaaaggaggactggaacggcctcagcctgaacggcagggattcgggggtaaagtagggctctgaccgatagggatacatggatcttccgcataggaaacgcagtagatccggatcgaaaagggccaaggccgacacgacccgcaggggcgaggggaattttacggagtagacgtgttcgcaggtgtcaccgaggttgtcgctgtcccatcttatgtgaaaagtggacgaataacgagagggagacgagatctgcaaagaaaagaaagttttattgggggataactttttcagtattcgggagagtagcccgcgcaagtctgacaaagcctgttttcgcgcttgcagtgcatgaccgctgcgcaaggtacggttctggaggtcgacgcgacaaagtcttttaattctctgcgggggttgtggcagacgggggtgagctcttggggagccgtgaggaacaggatggtcgagtttctgcacaggaacgaacaggcgatagagacgtcggtgcaatggatgagcatttggggcgctctgacgaagacggggcgaccggcgatgtagcaggtgcccgaattgccctccataaagtgtagcgcgagcgtggacggggctctgtcgacgaagggcacgcagtagagcgacgtgtgttgggcgacgttggctatccgctctatgtcgttgagatcgctatctgagatggccattgggaagcaggaggcgaggacgttgtacagcagcttggcgttggcgaggcgtcctccgcacaggatgagcgtattgatctctccgttgagccaccgtttgatggtgagggcgcacagagccgcgtcgtacccctctttttcgagcagctgatggaaccagttctcttcgggattgtagaaagcgagtctgagggactcgggttcctcgtagggcagttgggcgtagagagatctggagtttccgaatctttctcggagggcccctaggacgtattcccgctcgtccggtctgagggtgtactggtcgtaggcgggcatctggtcccactgagatcggtgagcgatgccgtctcggaaaagccgttcgatgagcgcgtccatctgcgacgccgacctgttggtctcctgagagtagcgggaaggagtctttttgttcggatcgggtgtgggcggagtttctgggacgtaaggaaagccggagaagtcgtcttcgtcgtcctccgtgcgcctcttctgcgacgggggcggcgaggagggagagggactacgatgttccgctttccgcttactctggaagagagaggatatgatcaaacttctgcttgcaggagtaacacgggggatcgatccaggcggtggagcagagcactccgaaatcgtttttgcagtcaaaatcgcgttccccttcgtgctcgcgtatctgcctcaggtattgcacgagctcgctggtgaggaaggagattccgtcgtcgttggcggtttcgaactggatgatgaggtggtactttgggttggtgggtagttggtctgggcgcggcagcttgttgagtcgcacgacgcacttcacttcttcgatttcgacgagttcgccctgatgcgagacgttgaaagccctgcccctgagcatttcgttgacgagtgggtttttaaaggggtactcgtgatgcaggggcgggaagtagatgagtttagtgacgtctcgcacgggaacgtactggtcgaaatcgaagttgttgacgtgcgcggtcaggacgcagtggaacatgcgcaagatagagttggtaaaggtgtctgcgcaggtggaggagtcgcccacaatgtagagaacgttgagagtgtcgtgcaagcgcgaaagcgtgtagtcgctgagccagcgaccgagcatgtagcttagggtgacgagattgaacccttccctttccgcgaatcttgcgagatgcctgctggtttctatggtgaaggggccgctagggctattgagtagggtttggtagaggctaaagttgcagtagattttcctggcttcgtggagaagcagttttccctgcagacctactccgtatcgagcgaattgctccggatccctgagacgccattctccttcggtgaaaatgagcctcttttggagctggtaggcgagttcgcccggattttcgggggcgttcgaccgcttattggaacccgtttgcctcgacctgcgactctggaggggaagacaggggttcgaagacggttagtttagggcgcttggcgagcatgtttttgcgagcctctgcgaatcgtatgatgagcttggaggctctgaagaatttttcctgcacgttgatgttaaggggcaggatggcgtaccgctgatcgagcacgcaccagcggaacgagtcggagacggggtcgggggagtaagtgagccagctgaacttttggttctgctggagaaaagcgaagtaggctttgagtaacacgaccagttctttgctgatgttgtgggcgtaagagtagagaaagcgcgagaactgaaattgggggatgtggcaagagaggatgtgtattttggcgttgaccttaagggtcggcacgtttcctatggcggtgcgcggcgcgagattgtggagaaccacgaaaacgtagaaagcggtacagttagcggaacgagcgaagagcttagaggggagagcgtgaaagagcacggagacgctagacccggagcagagtttatccatgcactcgtccatgacgatggccagcggtccctgccgggacgcgttgacgtatacgttgtccgggtgttcgatgttgaggttttcgggcgaggttgcttcctcgtacgtcatttctacgaactccggtcggaaggtgcaggttctgggcgcgaaggttccgtcctccttgcagtcgtagttggattccagaagttgtaggttccaagccgtttgttccaccggcgggatcatattcttctccggcgtcacaaagataaccgtttccgggatcggttgcagcatatcgcaggagatcaacgctctgagcagatggctcttgcccgatcccgtcgggccgtagatgacgccgatgacgggctgtcggcccatgttgagcgacggtagttgtccgtcgacgaggtaccgactgtcttcctgttcttgccgttccacggctagctgtatttctaggaacttgtcgtccactcccccgagactgtaaaagtcgtcgaagctgggaaatttctgttcgcgaaagagatgtggggctaggtccgccgctccttcgtaccagcccgttacccgtttgtagaactcgcctgcccgtagatactcttcctctcggtagcgccatgttttcctctttttattagcgacggccccggcctccgctccgctcatgggtctccgaggagatccaaaatttcgtcacagtcctcgatagagagcgaccggtctgggacgtcgaactcgtccgagtcctctccgtcgtcctcgggagcgatccgtgcggccgccgccgccgcgagcagcctgaggggggctagaggttcttcgtggcccaccgggggcactctccggacttcgtcggcggttctcgggttgggatgttcggtgtcgtaggggtaaagaaagtccccgtggcgatactgcgtgaggtccttccagggtcttaggactctggtgagctgttcgttgtggatggtgaacggatcgtatcggctcaccttgttgaggagcgtggttttgaagatggtcctgcgcgtgtgaagctcgggaatggcgctgaccgcgccgtacgactggtcttcgtgcctctgccagcagcgttccagcgtgtcgtatataagctccgcctgtctgtgtcccttggagcgtatttttccgcttcccacgtgaccgcactcggggtcgagacagacggcgtctttgagtccgtagagcttgggggcgaggaaaatggcttcggagctgtacgtgtcgccgccgcaccgcttgcacttgatgtcgcagtcgcaggcccagtagagcgccgggttctccgggtcgaacgtgagccgtgtgtgcgggcccttgatgcggtgcgcgcccctctccttcatgcgccgataccccgactcggtgacgaagaggctgtcggtgtccccgtagagggtctgggggtccctttggagtaggtgtgtccccctatcgggtccgtgcaggatttcgcaccactcgctgaagaaggcgcgcgaccatcccaacacgaagcaagcgatttgcgtggcgtatctcttattttcgaccattttgtctaaattttctagatgtagaacggtcaacgcttcggggggagcgtcgagcaaccgcatgggtttgaaaacggtctcgttggcggtggcgtaatgggcgtggtcatcctcggctatataagggggcgcgtcgagcgcttcctgcagttggtgatcgacttccgccagggacgcttcgcgagcggtaagtgcgttttcgagcttactggtactctcgccttcgctctcttccgtttcctcctcctcctgctcttcgttttcttcttctgctgtccgcgtcgggggtttccggtcaaagtactgacgcagttgatgatgtctgaaggcgtcgggggtgctttcggggcagacgaccgtgcccgctagcgagtcgtggttgagcaatgtcacgtgacgcacgatttgagtgccttcgtagatgccccgcctgtcgtcctcggtgaggtcctgttcgaagaggatgcgcgtggtgtccatgttggtggcgaaggcgccgtagagggcgttgcttagcattttcgagatggaccgcataacttcgtttttgtctcgatccgctttctctttggccgcgatgtttttgctgacgtattcagcgcagacggttttccaagcggggaacacgatgttcatgtcgtcgtggagggccgtgaccgcccatcctcggttgtgcaacgtgaggatgtctatgacggtgatgacctcgtcgtacagcgcttcgttggtccacacgaggcgcccccctcgcctggagcaaatgggaggcagcgtgtctaagtgttccgcgggcggaggataagcctcgacttttaggatgcacggtttgattcggtggtcgaagtagctgatgggtcgttcggaactcatgagctcgttgagctcgtcgacgtgtttggcagtgaatttggggtccaagggcatgccgtggggcatggggtgggtgagggcggaggcgtacataccgcatatgtcgaaaacgtatacgggatgtctgtacgggcctagcacgctgggataacaccgcccccctcgcaacgcttgccgtatgtatttgaacatgggacggtgcggggcgtatatttcggcgacgtactcgggggagggaagcctcttttttctttttttggtgtttttgtttgcgcttgcgcgctcgacgtcgtgtacgtcggcgtcgtgagggttccccttgatgtcgtttttcttgagcgcgacttttcttttgtacttggaaggggggcgctcgaccgtgctcgcgcgttcctgctcttcgacgtacgcggtgaaggtaagttgcttccaaaaggcgtgggtgttgctgggaatggtgggtcgcaggaaaatgttaaagtcgccgtgcatgccgagttcgtctttgaagtacttgtcgtaactgtcgtacaaggtgagagctaatttctgcgtgacccttacgtcttgcatgcagtactcgaggcacgcctgcacgatgtcgtacggacgacccgggtgctcctgtcgccatagcgccttctgttcggcgatgacagaaggatcctcccagtatctcgcgacggggaacccgtcggagtcttgttcgtaaccgccgatggagacgtgttcgttgacggcctcgtaggggcactggcctttggagagctctagggcatacgcggcggcggctttggagagtttggctccgctggtgaactgcaacgtgtcgcgtaccatgaatcgcacgaagacggtgcgggagtcgctgggcgcgacgactcctcgcgcccacctgtgaagccgcgtggggtcctttttatcgtagttggggttgggcaggtggaagaggacgtcgttaaagaggaggcggcctacgcgcggcatgaagaagcggtcgcaccgacacgcctgcggaaagacgtcgcgccgttccacgagttcggtggcgagcaagagctcgtcgaacttgcagatgttgtgtccgagcacgacgatgtgaacgttgttaaagtcgtcgggcagtttgagaggttcggtaggtttgtcgaacagttcgtaggggatgtcgtagcgggaaaggtatttgccttcgctcatgagcttgctgacgtagtctccgttggctcgacagtacctgtccacgagatccctggcgaagtgttgttgcaaacgggaccggtaggcgcggaaccgccgggcaacgaagccgggccgcgtgtctagccagtagaagccctcttgtaaagtttttacttccgggtcaacgagcgccaggtccgtggccgcgcgcacgacgtcgggatcgcccgtgagcatgaaacacaacataaaggggtgcatacgttttcctttattttcgaagacggtatacgtctcgatgtcgtaggtgagaaagagttgcttacagtggggttgctgagcggggcatgcgaaacgcacgtgttgccacaggtcgcagccgaatttttggaccgtgtggtagaaaaaggcggaccgcctttcgttgcacgtgtgattgcgcacccagtggcgtccgcaggcgggacaggtttgcacggccgtgcggctgagtatccaaacccagtcgccgttctggtcttgggtgaccagcatggggggaagaaccggatctccgcgttccgcgacgcgtttgacgtgcgcgagacgccctcggaagcggacgacgccgacgtaagcgggtttgaagacgggcagtctttccggggggttttcttggtagtacccgtagtctattctatcgtatccgcggcacctgcgcgtgcctgccgtaggaacttgtgtagtcgcaagaattttttcatgcctttgtggaacacggccggttgcagacggaacggtacgccgtcgatgtagtagacgttggcgcggatgggatctcccttggccgccttgaagtgggtcttggcatcgttttggctgagcgtcttaaccaacggcgtgtcttccggtccgagcagagtgttttctaggggaggcggggagtacgcggcacgggaagaggaggaggcagacgacgagaggctcatcgcatgcgaggaggcgcgtgccgagcgacgaggagttcctgttctcggtctctcaggacccgacgcaggttgtccgtgatggcctcgttggtgctgatggccacgatgccccggaatttgatgcgaaaactgatgtcgatggagtcgatgaactcttcgctgagattgagttgtttgaggacctcttcgatgtcaccggaacggtctctgtattgaatatcggagagaaataagtgttggtctgcttcgtccatgccttcgaactgccccgtgcgctctatcatcatgagaaaatcgcgcaggatgcggttccacagggtttcgaaaatggtcgcggggttagattgttcgctccagatgcgtttgaaaataggctctgcgttgacgtcccaccccacgatcagtacctgcagggtggtgacgtctacgtaccgccggaactcgcggttcgcgacgaagtgcgagtaaagatagtagagcgtggaggcgacgtgttccgcgaggaaaaagtagagcacccactttctaagaaacgattcggtgacgagcgccacgtcggcgtctcgcgtttgtaggagcagtcggtaaaagctatccgtgaatcggaacagctcgtgtctgcgggcggcgccggagagttcgttttgcagggcgtcaatggcttccagcacggtgcggatgacttcgtcgagcagcgtttcttcttcctcttcttcggggggcatttcttcctcctcttcttctgggaaggcttcttcttcgggaggggccgggggcggaacgacgcgtctccgtctgatcgttcgcggaagacgatcgacgaattcgcgtacggctctccgcctgatgcgcctgacttgcgaggcggtgatggctcgcccttgtctgtccctgggtcgtagcccgcgtctgtcggggacgcgtctgttgcggaggacgatggcgccgcccgagaagggatcgcctccgtccccgccaccgccggcgcgccccgcgtaccctctgcccgaggccagagtgctaacgaaacatctcgccatggtctccgcaggttcctcggcgttcactctcggatcgagtgccgcttgtcggatcaaactctgcgtgtctagatcggcgaacgccgcttcgaagagcgtgagccagttttcttcggcgaacacatcggatccaggtaagaacctatacgtgttttccgtattaaaatgttcgcgcgcgtaacagaataaatagtggcacagagcgactcgcaaacgccgtatcgcttccaataaggtcgcgtcgtctctcgacgccgcacgcatgataatgtcgttttgcaaacctcccgcgccgctacccgagaggtggcttcgcgcagcagcgagcgcggcgtccccgtccttcccgacgcccacgacctccccggagcgcgcgacgtcgaaccctctgcctcgcagatgaacgtgcgccatgtcggaggcgattctgtccataagcacggcgttgtgcatctgctgaaagctgtcgtgaaagttttcgaggtccaggaacctcatgtacgcgcctacgttgacggagtacgagcagtcggtgaggcacgtccagaaaagcctcctgggtcgctgcgcgggcggactttcgtagccgagttgcatgaagacgcgattttcgaaaaagtaatcgttgagcgcgcggtgcatgtactggtagccgagcaggaggtgcggcggaggcagtcggtgatacgggtatcccgcgacgttgggtccgttcgggctgaggtccctgagctgcatcaatctgtagtcgtagagtcggctgacgagaaagacgctgttggggtgtaccagcgccggctgattcctgaccatgggaaagtcggacgcgataacgggttgacaaaatcgaacggtgtttaagctttgaccggtgagctccgcgaagactctgtaagcctgaaattgagccctgacgtttttagaggagggcctgttcccaaccgagagacgccatgcacccggtactccaaaacgttcggaacgcgagcgcgggcgccggcggggaaggaccacaccgtcaccagcatcagcagcaacacgtgcaacgccaccaccagcaacagcaacggcaccgacagcagcttccgcaagcggcgccgacgcgaaaccgcgtccgccctcccacccctccgcagtacccggcgcagcacgcgctgccctcgtccgcttccgcggacggcttcgcgtccgacggcggcgaggacctaggtcctcccgtttgcgggctggcggcgggagcggacgtagacgagattcgaatgcgaaagcgggaaagcggtcgccgcggagcgattcccgagacgaatttgtttaaggcgagcagagaggcggtcccgcaaaacgattacgatagggaggcgatgtaccggtcggggcaggcgatcagcgttaaccggggtcgcgtgctgaccgccgacgacttcgcgtacgatgagggacaggacccgtcgttcacgccgggtgcgaatcacttgcgcgcggccgagcttgaaacgcccggccgagcagaccgcgttcgggaagagctgcgcaacagctgccaccaaacgcgtttgcgtacggcgttgacccgtcccgagctgcccgcggggatctactacctgtacgacttcgtgcagacgtacgtcgatcatcccgacgggcgagttaagttaaacccgcagctggttttagtggcacagcacgcgggcaataccatgctcgcccaacggttgtggtcgatagcggaggataagaacgcgtggttgcgtgacctgatcgagatggcgtacatgatcgtgaacgatccttacttgagcaccgagcagcaattgtcggcgatatgcacgaccgtggtggagttgagcatgaaatacgctaagatcgcggcgacgaacggttatccgtcgatggcgcagatggctaaggcgcaagaattcttttaccgcgtgatggaagccgtgttagacttgggagttcaggttggggtgtacaacaaccgtccggtgcggttccgtcagaagcgcatcggcgagatccctcagatgtctgacgcggactacatgttcggtttgacccaggcgctcgagaacaggcctcctcagggcgaacttttcccgtcggacgagggagaatccagcggcggcgaggcggaggaggacggctacgatgacgactactgagtcgtttatgcttttggcccctctgggtcgcgaggaagtggcggacgccttaagctcgtgccggacgggccgacggcgcgttcgctttcgccatgctccgtactcgaaccgtttgcttaagttgcaaacggcgatggttccgccgaagatagacggtacttcggaacgcgtggccgaagtggttaggggtttggccgagcagggcgccatttatccggaccagatgggggccatacattccgatctgctaaaccgcgcgtacacgtggaactcgatgggagtgcaagagagcatccaggccttggtgaacgacgtgattcacgggcagaacaaggcgctgcaagacgagctttcccgtacccgcgagatcgcgaacgcgtcgctcttgacccaatttttcgatagcatttacaaaacggtggacaggggccagcgtaactttgagggatttaaaaagctgctgcggcttttcgttaacaacgtccctaacgcggaggtgtacggctcggggggttcgttcagcatgcagatcaacctcggaggcacgagccagaacatcaatttgactaacgcgttcgaaaacttaaaggacatatggggagcgcgttgggacgcggtaaacaatccccggataggagcgctgctcacgcccaacacccgggcgttactgtttttcgtgagcgccttctacgattacggggctatggagcccggcagttacctggataacattctgagattgtacaaagaggccattagggcggacatagacgcggagggagacgccgtgatggagttgggcgaagcgggagccaacctaaatctgcagttcaacgagtacaaggataccctgaactacctgcttcagaacagacagtcggtgccggatacggcgccgctcgaattgagcgaagagcaggaaatgcttttccgctatctgatgcgtcaactaaggcaagcgctgaaggacaggattccttcggacgtttccgtgagcacgatggcccaatacgtggacccgcgcctttatcagacgaataaggtgtttatcgaaaagcttcaaaactacctgttggccgcgcacgcccgcaatccccattactttagatcgatcgtgatggatcgagactggcgtcctcccgccgggctctacacgggtaactacgtcataccggaacgcctgccgttcgattattacgacggcgacagcgtagtcggaggcccgtcgcgagacgagtacttcgaggagtatccctacgcgagcaaaccgtacaaaaagatgagcggtcgggagagggccgactaccaggagcagctggataacttaaccacgcagatagatcaggctttgggcgtgcaatcggaggccggatggttagccgatcaccgcttgccccaagcgttcgatggtgctttgagtctagcggatctggcggcgatcccgttacccgccagtccctccgatcaatcgatggcttcgagccggcgtagctccctgtcgagcgtaggcgacatgatgtcgcgcctgaacttatcggggcgagggggagcgggattttttgcgagcctcagaccgaccttaggaagccctagaccttctagcagcgccagacctagcggattagcgttgggcctgaggggcacgggtcctgcgcgcgcttacagaacgcctcgcgtcggcggcatgtcaggctccggattggctagaagggctttggcgacgcggtctatgcgcgacgggaaaaggctgcggttttactagcgtagatgcgtagaaacggaagacgaagaaggaagaatgcgcgaggtgtaacgagggaacttaccgccatttctagagcgatgcttggtcaccacgactttggtttccgcgaagcggcgttgaaccggggttcctcttcctccttcgcgacgtcgatgccggccgctcctcctccttcgcctgtgtcgggcgtgccccctgcgatggctcctcaacgctacccggcgacggtgcacggataccctccggtgattccgccactagactcggccgcggacgacacgtccgaactgttcgttccggtgcagagggtgatggcgcctacgggtggaaggaacagcataaagtaccgcgattacgcgccctgtcaaaacactaccaaattgttctacgtggacaataaactgagcgacatcgacacgttcaaccccgaggcgaatcacagcaatttccgaaccaccgtgatccataatcaggatcttgatccggctacggcggcgaccgagaccatccagctggacaatcgatcctgctggggcggggaattgaaaaccgccgtgaaaaccaattgcccgaacgtcagttcgtttttccaaagcaatacggtgcgagtaaagttgatgagttaccgcgatccggtgcctccaggcacggcagctcccacgagccccgagccctacgctccagccggtgctcagtacaagtggtacgacctaacgattcccgaaggcaattacgccttacacgagatcatcgacctgctgaacgagggagtcgtgcaaatttatttaaaagagggacggcaaaacaacgtgctgcgctccgacatcggcgtaaaattcgatacgcgttactttaacctgcttcaggacccggtgacgggtctggtcacgccgggcacgtacgtgtataagggctaccatccggacgtggtactgctgcccggatgcgcggtagactttacttacagtcgactaagtttaatgttaggcatagcgaaacgcgaaccgtattcgaaagggtttctcattacttacgaagatctcgaggggggtaacgtgcccgcactgctagacgtggaatccgcgcagatgaccggcgtcgatcaagacgtgatcgagctggcggacgcgaagcccttgttaaaggactcgaagggcgtgtcctataacgtcatttacgactctaacaaccgtcccgtgaccgcttatcggtcttggcttatcgcgtacaaccaatcgggttctacggcaaacgaaacgaccttattgaccgttcccgacgtgggcggaggcataggagctatgtacacatctatgccggatacgtttgtggcgcctaccgggttcaaggaagataacacgacgaaccttgccccggtggtgggcatgaacctgttccccgccctcaataaagtttattaccagggcgcgtccacttacgtgcaacaactggaaaattcctgtcagtcggccacggccgcctttaaccggtttccagagaacgaaattcttaagcaagctccccctattaacgtgtcagccgtgtgtgataaccaacccgccgtcgttcagcagggggtgctcccgttgaagaattctttggccggcttgcaacgtgtgctcattacggacgaccaacgtcgacctataccctacgtatataagtccctggctacggttcaacctcgcgtgttgagcagctccactttacaataaaacactcaaaaatccaaaatcgtcgccgatcgctgaaaaccatgtccattctgatctctcccaacgacaacagaggttggggcatgcgtcgccgctcgtctatgcgtggggtcgggattcgtcgtcgacggttgacgctgcgtaccctgctcgggctgggtaccagcagccgacggagaagcggcggtcggtccagcagacgccgttcccgccccgcttctaccactactcgcgtaatgctggtacgtaccagcccgaagaaggagacgttaacgcgcgaggtcgactggaaaacgcagatggaaggaggaggaatgaaaaattgaaggaggaggaggacgaggacccgccgttcatttttcttgactgttgttttaacactcgtaatcggctgttacgcgagaggcttgtaaataaatggagagaaaatttgcgcaacggaatgagaaaagactactgatttgcctgtaccgtcgctgtactacgcaggaagcgtcgccaacatcatgccggcagtagtgcttacgggcgggcgaacagctagagctaatcggagggcgtcaaccgcttcccgccgaagactccctgcttccaagctacgggccacccgtcgaacgcgccgctcagtcaacggtagtaagaaaaagcgttcgccgaacgtggctgtggcggtaccgtcgcccactacggcctccgctgccgagcgagccgcgctgcagaacttagctacgcggttacagcgagggcagtttacggcttggcgttcggcgaactaccccgcccctgcggcctccgaggccgccctggccgctgctcaaagcggcgcacccgctacggccagggacatgacgaccggaacgaccgctacggcggttcccgtttcaggtgccgggatcgcgtgttcaacgaggagaaggagaaacggtgttagcggcggtagaacgcgtcgccggggaaaacagctgaaagggggaattttacccgctctcatacccatcatcgcggccgctatcggggcgattcccggaatcgccggcacggccgtcggcattgccagtttgaaagaacaacagagacagttcaataagatgtacaatcagaagtaagagagagaaaagaaaaaaaccgcgggtgccggtgctgtctaaaaggccgttttcaataaaaatttttatagaaccgctgtcgccgccgtcgtttgccgtttgtcgtcgtcgtcgtcgtgagcagttgtcatggattacgccgcgctttctccgcacgtcggtggttgggccctgcgagacggatacctcggagactctagcctgcgagggggtgctatcaattggtcgaacgtgggctctcgtctctcgagcgctctcggcacggccgggcgatggatgtttaaccagggaaatcgctttctcaattccaacacgttcggccagatcaagcagggctttaaggacagcggagtgatccgtaacgtcgcaaacctggccggggaaaccctaggcgctcttaccgacataggtcggttgaaaatacaacaagatctagagaagcttcgccgtaaagccctgggagaggacggacccgccactcaagccgagttacaggcattgatccaggcgttgcaagcccaagtcgccgcgggggaatccgttcccactaccgctcctacggtagggccttcggctcccgccgaagtgcctcgaccgacaacacgccccatccccgagatggtcacggaggtgaggcctcccgtgacgtcctcggctcccgcggtgcccgaaacggaccggccgacgaccctcgaaatgcgtcctccgcccgcgaagaggaggagaaagaggccagcccccggatcgtggcgtactcgcctaaacagcctttcgggaaacggggtcgcagttagccgccgtcgcatgtgttattgacctctcgataaaaaagcgtggagatgaaaaaggcattaaatcgtatctatcggattaccaaaaatttagcatgtcgccgtttttttaggtcgatccgccgtcggctgccgctatggccgcgtttacacccgacctgaccaccgcgaccccgcggctgcagtactttcacatcgccggtccgagcacccgggaatacctgtccgaggaccttcagcagtttatcgcggcgactggaagctactttgaactgaaaaacaagttcaggcagacggtagtcgcgcccactcgcaatgtcaccaccgaaaaggctcagaggcttcagatcaggttttacccgacgcagaccgacgacacgcccaacagttaccgcgtgcggtacagtttaaacgtgggcgacagttgggttctggacatgggagccacctacttcgacatcaagggcgttctagacagaggaccttcttttaaaccatacggaggaaccgcatacaatcccctcgcgccccgcgaagcctttttcaacaattggcttgagtcagagccgaacaagaccgtcattacggggttaatgaccaccccctaccgaaacgaccaggggaacaagaccaatactgctgacgtagttaatagcgtgtcgggagtttatccgaaccccaatctcggaccctgcatcagcgagatgggagcactggatgatgcaactgctgaccttgtcggctttgcgggacggtttgcgaaagttacaaacgagaatacgcgtttggcatacggagcgtatgtgaaaccgttgaaaaacgatggttcgcagtcattaaaccccactccttactgggtaatggacaagactgacgccaagtatctgggcgtgatggccgtggaagaattcagcaccagtctcacctatccggacagcttgttaatccctccgccctcggactactcaaccgttaacacgggcgcaatgaaagcaaaccgtcctaactacatcggtttcagagataacttcattaatttgctatatcatgatacgggcgtgtgctcaggtactctcaattccgaacgctccggaatgaacgttgtcgtagaacttcaggacagaaataccgagctaagctatcaatacatgttagctgacatgatgtcgcggcatcactactacgctctgtggaaccaggcggtagatcagtacgaccacgacgttagggtgttcaataacgatggctacgaagaaggagtaccaacgtacgcgttctctcccgagggcacgggatatggcgctaatcctaattctaacctgtcgtttgctgacgtgaaagtgcatcaaaacggggcgggcgacaaaggaaacgagattaacacgggaggtgcaacttactctacatacttaaccgtgggaagtgtgccatcttatgaaatcgatcttgctgcttctcagcggcgaaacttcatagtgtccaatattgccgattacctgcccgataagtacaagtacaatattgatggttttaatcccgagacgggtaacgtagaccctactacatacgaatacatgaaccgcagggttccacttaccaatgtagtagatctatttacaactatcggcgccagatggtctatagaccagatggacaacgtgaacccattcaatcaccatagaaactggggtctgaagtataggtcgcaattgctcggtaacagtagatattgcagattccacattcaggttccacagaaatattttgctattaagaacctgttgcttctccccggaacttacacctatgaatgggtgctgagaaaggaccccaatatgattctacagtccagcttggggaacgatctgagagccgacggagcctctattgtatactctgaggtgaacctaatggcgaactttatgcctatggatcacaatactagtaaccagttggaattgatgatgagaaacgctaccaacgatcaaacgttcgcagactacctgggagctaagaatgcgctttaccaggttccagccggctccactgcacttactattaatattccagcgcgtacatgggaggggatgaggggttggtcttttacacgtgtcaaagcctctgagacacctcaaatcggtgctcaatatgatatcaacttcaagtactccggttctattccgtactcggatggtaccttttatctcacgcacacgttcaggaacatgagtgtattgttcgatacgtctatcaactggcccggcaatgatcggcttctggcacccaatctattcgaaatcaaacgtaacgtcagcataaatgccgaaggattcaccatgtcccagtgcaatatcactaaggactggtatcttatccagatggcgaccaactacaattatgtatttaacggctacaggttctggcccgacaggcaatatttccactacgattttctgcgaaactttgaccccatgacctgtcagggacctaacttccaagatcaaactttatttgatctcatgagttacgatccagtgcagactcccggagccgttcagaccaaccaagacgctatccgtaacaattccggttacacggctcctcgcagctggccggtatacggagcacaacagggagaatcgtggcccgcgaattggccgtatccgcttatcggtgacagctcactcaatcctacccagatagtaaattacaaaaagtttttgtgtgataattacctgtggaccgttccgttcagctcggacttcatgtacatgggtgaattgaccgacttagggcaaaatcccatgtatactaacaactctcacagcatggtcataaatttcgaactggatcctatggacgaaaatacttatgtatatatgctttatggtgtgttcgatatggtaagagttaatcaacccgaacggaacgtgctcgccatggcttacttccgtacgcctttcgctacaggcaacgcggtgtaaaaaaactgattaaaaaatgtccgggaccacggaaagccagctgaatcaactagtcggggccatgcacctccgccatcgattcctgggcgtcttcgacaaaacttttcccgggttcctcgatcccaaccgccctgcctcggccatcgtgaataccgggtctagagcgaccggaggtatgcactggatagctttcgcgttcgatccgatcgcgcgaaaatgctacatgttcgatcccttcggttggtcggatcgggaactgtggaatttgtacaaagtgaaatatgacgcttttctcagaagaactggattaagacaacctgataaatgttttgaactcgtacgttccgtcgaagcggttcaatgtccgtgttcggcggcgtgcggactttttagcgctctttttattgcttcgtttgatcgctaccacacccgtccgatggatggtaatcccatcatcgatacggtcgtcggcgtaaaacactccgacatgtacaaacccgaattccagagcattttgcaccggaaccaggagcgaatgtatttctggtttatgaaaaacaactctttttttcgcgcacacgaatcggaactgaaacgcgaaacggccatcaacagcgttcccgaaaaccattaagacattacactcttgtaaatttctatatctgtattttttattttcgcattcgcgacaataaactacatttattttcgagaccgcgtgcgattattgctctcgtccgcgcccgttatgcgaacgggtcgcctgtttcaacgggtttaaccggagcgatgacctcggttttaaacccgaaacgctcgtgccaacggaattcgggaacgtgagtcggcgcttgaacgcccatggcgttcaacactaattccgtggcaaaaacgtaagcgtggcgtagatccatcgcggaaagccgccaagcgcaggttttatcggaggtcttgcgaccggagcgagaggtgggaccatccgtgcccgagggagattgcggattgcagcacgtgtacaccatggtatgcgggtacttcttgtgcgccttcatatcgggacgcgagcgagcggtatcggaagcgatatcgtcggtgccgctcagcttgtatgggatcatgcgacaaacctgacgcccgctgatgggaccttgaacggcgtaattacaattacagttggtcgatatcagaatatgctcttcggcacggcgtttttccgcatttggatagagagccttggtccactctaagtcgtgtctcatggcgctcaccgctttcgcggcatccgagaaggccatgccgcagcttccaatcacgtgagggtacgggaaaccagagtggtcggcgtccctggagcacacggcgttacggtcgaaccgcaagacgaccacttgtttaccgaagcggttcttctcgatttgaccgttttgctccgcaatggctctctttcccgcttcgctagtagggttgagctcgacggtgcgcggcttcaagaacatggcattaccatgcaagcatttgggggtggtgttggtggtggcttcccatccgtgtcgccatacgtgcgctccttccggaacgaacttcggttcgagctccgccattccgtacaccatggccgccagaaaacggccaacttggttgtggaaggagtcgaaactcgagaaggtaagtctaaactcaggatgcctcttgcgcacgaatgtacctccaatcctggtccaaatggcatcgtcggggcgaatagtggaaccctgccaccggacatcgagtcggtcgcaaatcgttgtcagaatcttcatggccttctgcgcaccgtactctacgggatcgcttaacggcctttctaattcttcatccgattcaacgtcgagttcggatttcttttcgtcgacttcttcccgttcctgcgtttccttgcgggcttttttgctgggcgcggcaccccgagacttagcgctcctcttctttttcgagtccaccatcgctggttcagcgttctcatgatcgtcgctagacgccatctttttggaggtagttttaggcgcggaatcctttaccatgccgctacgatcggtttctccttcttcctcttcttcgtcctcacccggtgagctctcttcagaactggagaatacttcctcgacttccagcctcctcttttgtaccttgacgggatgacctattggttgaacgaaaccgttttacgacgacgtcacagacccctcccatagcccccagcgcggtataaaagtagatttccgggtcggtacgaccactcttatgccatcgagggaggctgcaggagcccgtacctcggcgatccgacggtggaagtgtctccttcggtagcggtgcttcctgcagcggcctcgtctttggttggctccaatccgattccgagtcgtccgaattgggcatcggagtcttttccctggctccgaatacctgtcgaatctcctcgtcgtcttcgtccgagctcactacccaaagatcgcggtctgctgcctccgccatcacggttcttcctccggctcctcctagagagttcagatcgagggaaggagagaaaacggcatcatgcaaacggctcgcgaagggaaggccacggtcattctgaatctcgtcatcaataccgcgaaggaaaaaatcggttggcagcgcttcgtggacgcgatccaacggtacgtggccgaagcttatggtgctttcttggcgctcgacccagaggcggcaccacctagacgcgaatccgaccacgcggtgcgagttcttatcgatgctttaggggaggagagagcagttttagctgcttatcgcgtggcggaggagttattagaagataaggagatgccaaaagaaagccaagacaaagaacctttgtctgaaaatgaggaacttgcgcattctttcgcggaaagtaccgtttctccgcattcttttgcggaaagtaccgcgacgggtgatataaacgtacccgatgacgagagttcagtcgcctcacaaacttactcgggagaggaacgggacgagtctgagtgcgactcggacgaagaagaaaacgacaaggaggcgaacgaagtcgaagcagacgaggcagaagagcaggaggaggaggaggaggaggaggaggaggacgaagaagatgactctagcccctccaccgtgctggaaaacgagcgaatacaagaaaacggggaacccgaccacaatcccaatggagacgagggaggagctgattctgatgcggatagcggatactattcggcggacgcgggacgattgggatcgttactttcggactcagaacacgaaaacgacaccactgaacggcaagtggaagtgggtatcgaggacgagtctcctactggtcaccatccacttgggactcctgattccgatcgcgatcatcaggagcaagaaacttctatagagacgaaacatgtagatcccgtttctacttttaaaaagtgcttcgaacgccaagctgctctgcttaccggcgcccttaagattccttgcctgctgaggacgccgacgaacccgtctccgtatccgcttgtgcagtaccagctagagagattcgtattcaatcccgacccaagggtccctcccgaacaccgcgaagtgcgctacaatttctaccctcctttcatgcgtccaaaagctatcgctaattatcacattttcgccgttaccgcccccatccctgctagctgcaaagcaaacagaagcgggagcaaattactagagtcctgccgacaaacggcaacgtttaagcgcttacctcggtggcggatcaacgttcaattcgatgacgggctcggagaagaggtgattcctgtaacagagctatcagatgcaaagttagttcctttgcaagaagacatttcgagattgcagtgggccaaaatgagaggtgaacatattcggttctttagctatccctctttacacatgcctcctaaaatttcacgcatgctcatggaaaccttgctacaaccatttgccgatgaaaacgataaaggcgaaggaccaaaaccgtgcgtgagtgatgaggaactgcgttatatcgtagatccggacggcaaaatgcgcggggaagaactctataaagctatgcagcggagacgaaccattgttaccatggcagttcgttttaccgcgcttctggaactcatggaacgcgtcctcagggagccttcttcggtcaaaaaagcacaagaggtgctccatcatactttacaccacggatttgtcgctcaagtacgcgaaacggctaaagttaatctgagtaattacgcgacgtaccacggaatcacctataacgaccctctaaacaactgcactgtcgccaagctctttgaaggtcgggacaaggaagattatgtgctcgacagcatttacttatttttagtcttgaattggcaaaccgcgatgggcatgtggcaacaagccatagacgacaccacaattcaaatttacaccgaagcttttacgcgccaacggagagccatttacgcgctgactagcgtcaccgaggtgtccaaagccatagtcgatcttctcatggacggggaccggttaaccgaagaaatgcgcaaagctctgcctaactttattacgcagagccagttgtctgactttagacacttcctaacggaaagatctaacgttcctacgatggcagcacccttctatccctctgactttattccgctagccttccgccaaagcgcacctctcttgtgggatcacgtctatctgcttcaagcggcttacttcctcatgaatcacggcggatacctatgggaaccctccgagagcgatgcggaatctccgcaatttagagcttactgtccctgcaatctgtgcagccctcatcgaatgttagcagacaacgtggctctgcacaacgaagtcctcgccatcggtacctttgagatcagaagcgcggatggtaaaacttttaaacttaccccggaactatgggcaaatgcctacctagataaattcgtggccgatgacttccacccgtttaccgtttttcactattccgaaaaccgctcatcttttggcaaaaactataccgcttgcgtcacggagagccccgaaatcctatcgctgattcgccagatacaggcctccagggaggagtttctgctcacccggggcaaaggagtctacaaagacccacaaaccggggaaacgctagccacttcggcggcgagcgtcggcgaggctcgacctggagctgccagggggtgcgtctttaccgtccgctcccaccggtgccagcggaggaactccagcgccgcaaaagcctcctagggctatacgggctgccgatcagatcatctccggagactcgcgacataccaggcgcgactacggggaaccgtctttatcaattccatccgactggcgatatggctcagagaatgctcgacgagaagaccagagtaaccgaagagccacccccgccgtcggaagagaccgacgctcccttccatacagacgggctgtacgcggcacgggaagcgatcgagtccgacggcgaaactctaggaagccaggatacggaggaggacctgagtaccatctcggaggaggaggaagaggagacttacgaggaagcggagaaggagaatatacctccgtcgaggggggcatctcgaaaacgccgctccgcatcctccctagagaagactctcccgagacctccgctgagaaagaaatcccgcaataacgctgacgagggtaatgcccaagggcttagaaaacgtcgccctagaggtaactatcgcagctgggtcagacaccgggtggctatctgtcaagctctacgcgatgcggtattcgaccgcaaaatggctgctgaaattctcaaaagagtgcacgggttgttcgtgcctcctactgtcttaggctattacgctcgaaaactcttagatcttaccgacgaagactctgatcgtcggtctcccttttttatgttcttagtgtccgacgatgccgtaatcgacgaagagccggttccaccgcctctacctcgtaaacggcgccgtagggcgaataaggaggaaccgaacgcctctgaaacacagcttcccgaacccgtatccccagcagtatctgatttgaaagccgaaatattgaatctgctcgttgaaatcgaaagtttcgtccgtaaaaacccgtcgcgccgcgtctcgattcgcaaccgtacccgcgagagcattacgcgccagctgcactacatgaaaagtgaacaaaaactcaccaagcttaagacagatgcggaaaaaatcctacacctgtggagatccctttcataatcccgcttcttttatagccctccgctgcgcttcaacatcatgaacctgctcgacgccacgcctaccgagtacgtgtggaaatacaacccgctctcaggaattcccgccggcgcgcaacagaattacggagcgaccataaactgggtggtgcccggaggcaatagtttcgcctacgcagcggatgagataaggcgaaacaccctgagccccgccgtcacgcgagcgataaccgcgcgcttcgaagctgaatcagaccagcaacccttcgccaacccccgggaaaccgcctacatcaccgctaacgtactggactctggctttccaaagtccgcggtttatcccgtagatccttccggagtacaaaaagttcagctcgctggaggcgccgaggggcgtatgcagctctcaggcggcctcactgaaggtcgagtgcaactttcgggtggtgtattaggacacgtgcctcgccgcagtcggcgaggcgccagacctcctcgatggtgcggaacagccctcgcgggaaacggactaccagaagacgccgaaatggtttccgacacctacaagtatttcctccgcactcaaggacccagccaagtggtctcagaaccgggcgtatactctcaacggcagtttatgacaacctttttacccgctgttgtcccacatccctttgacagtcctaatcctaacgattttcctgctcaatatagtgccatctacaagggcacaaacgcttatgaggatgtattttgggactggtaagccggtcttcacacttacccgctgctgtcgatgctcagtttcgcaataaagttcctccaattcacgttcgttaaacggttcccgtctcgtcattattacccgttcgccgccgtcgctcgctattcgcgctctaaaacgtcttttgagccaaaagacgtaaccggggttcaggggttgcgtaaatctaacgatcgcctgatcgttgattttcaaccaatattttttaggagcatccacttgcgcctccgacatggcgaaatcgactcctttcgcgttctccatggggcagcactccagccgaaaacgtcccgcggacagcgaaaacacgcaaaatgcatcaaaagtcgccaaaacgcagacttctgccacgcgcgccggtgtcgacggaaatgacgacctaaacctggtgtaccccttttggctccaaaacagcacttcggggggcggaggaggaggaagcggcggaaacccctccctaaaccccccttttatcgaccctaacggacccctctatgttcaaaacagtctcctttatgtcaaaactactgcacctatcgaggttgaaaacaagtcactcgccctagcttatgactcctcactggctgtggacgctcaaaatcagctgcaagtgaaggtagataccgagggtcccatcaggatttccccagatggactcgatattgctgtcgacccatcgacgttggaggttgatgacgaatgggaattggcagttaaattagatccaaacggacctcttaccgcttcatcagcgggaatcaatataaacgtagacgatacccttcttatagaagatgacgatgctaatcaagcaaaggagttaggcgttcatctcaatcctaacgggcctattactgccgaccgagacggattagacttagaaattgattcacaaaccatggttgtcaaggacagcggaacgtccggcggcgtactcggtgtattattaaaaccgagtggaggactgcagtcaagcattcaaggtatcggagtagcggtagctgatacgttaaccatcacgagtaacaccgtagaggtaaaaactgaccccaatgggtcaataagctactctgctaacggcattgccgtaaaacccgatccctcaggaccgctcacttcctctggtaccggactatctgtggttacagcagccgagggttcaatccaatcttccaatgccggtttagcggttaaaaccgatccaagcggaccgattaccagcggttcgaatggcttaaacctgtcatataatgcatcagattttactgtgtcacaaggagtgctaaacattattagaaatcccagcaccctccccgatgcttatctggagtccggaaccaactatttgaataattttacggcacaagccgagaattctagtgtattcaaatttaactgtgcctatttcctacagtcatggtattccaatggcctggtaacttcctctctctatttaaagatagacagagctcagttttcaaatatgccgacaggtcagtccgcggaaaacgccagatattttaccttctgggtacctacctatgagtctctcaacctgtcacgggtttccacccccacgatcacgcctaacaccgttcagtggggcgcattttcgccggcccaaaactgctcaggtaatcccgcctttcagtacaatctcacgcaaccgccaagcatctattttgagcccaaatcgggttccgtgcaaactttccaacccgtattgacaggagcttggaataccgacacctacaacccaggaaccgttcaagtctgcatactgcctcaaaccgttgtgggaggccagtcgacctttgttaacatgacatgttataacttccggtgtcaaaatcctggaatattcaaggttgctgctagtaacggcacattcactatcggacccattttctactcctgcccaaccaatgaattaacacgacccacataataacttacacgtgtaaatcaataaaaaagaatcgatgtaaaatctttattgatttaatgattcattgtcgcgtcccattcggcacattgccagtaatacagacaattgacagcctccacgaaccacgcctcactaattaaatgcaccttctgttcaggaaaatccacctgcattcttcggcagtagtgacaagggagtgcccccatttgtccgagcgttgctatggcttccacgaaaatattaactttattggggggaacgtaaattaccattcccagaactgcaccagaagccggtgaaggacaaaacaccggataaaaatcagtaaacatggctgcagcccaagccgccacaaaataaactccctcaagcgtgggatcatcttctaagcggctccacaaataaactcccagacctgtcccgtcgggctgacaacacacccccatgggaactcttttcatatcgaatccgtgacaatcacatttctcagtaatcaactcaaaatcttctaaacacaagaactgataggcatgtgccgcgggaacaaatcccacgttgtttacggcggcgggaacatcttgtgcctgttcagcaccatcagcatctgctagcgctctctcggccatctgtcacacttgaacgtcctcgatttcggcgtacgggtgactgtcctcggttaacccctcgctaaaaacgaccaatggaacgggaacgggaggagtaggatcggatggtagccgatacaacacggagcgcaatcccgcttcccctgaatacagggggttactgctaactgtccaggtaggagatcttcgtggaaagctcgacagtctacgcagccacgaatgtcttcgagatggtgttctattggacgcagtacgctgccttcggtcccgccttcccgtagcacaccaaaaaatcagcaataaactcacggtagttgctgtcaaaaaggtgcaacatccaaacacggtaaaaacaaaggtcagttcggatatacggtgactcaggaacagatagctgacaaccacggaagcgcagtaagaacatactactgctgaaatgcagaacaggatacatagtcttctgatccgagcgtcgctcggtacctaacaataaaagaaaggcgattttctatcaccttctactctagcacgtctttttgacatgcaattgcgtaagtaactgagttgtgcaatataagctagtggcaacggttgcttgaggggacaccccgggcatgcgctctcaggatgatgatcgcaataagtaccatgcacatgcaatacccattcctccacctctctataggtagcccgtctaaaggcgggaatgtaacacaaccccttagaaacaataggccaaacagaagggtcggccatctccctcaacattgatcgtgtcattaacggttgagtcacgggactaccactgccgctcgtttttaaaataacagtagctacaacattggtacggcatgcgcccagaaaaaggacaggatagggcaagaacggtaactcccttggcacctttgtcgtagacacctcgtaactaacagtttgtaacgcgaacttaaaagctaaactgttatctaacagaatccctgatcgcaaaaatacaaaatcggacttgtgtctcctgataatccacttgcgatgcctatctaccaactcggtcttggcagcaaaaagccttctcgaaagaacccgtaaaaactcctccttctgatcgggatccagttgcaatcttgcttgaacccttacaatcacgttcaagatgatcctcggccccgactttaccctcacatactttgcacatctacaactgactacggaatacagggactcgtgccacagataatgttgtggcttttcgaagaggtccatgctcatgattgtccgattcgtgtgaaattccatcatccgttctagggactcctgagtcgcaccctgtctcatcagtagactaaaccatatcactccgcactcattttgaaatccgcagcccctggtaagggctaccacctcctgtagaattacaaggatgcaagatgaaatcagaatatagagaagaatcagcgagcgcatgcagcacatgcataagcacttccatgaaactcaccgactcagtacacagaggcatgatgtcgagactgatgattttttattgatcaagtaagtccacctgaaacatattaaacaacatcataataaatatcgcggtaacatttacaacggtgatggcagaatatatacatcacgacacatcccgtgaaacacgcagcggctacaccgcccgtcacaaccgcgatacgcgtaactctatcttcccaaaattcacggatcagagtgtaaaactctcctccgagatgagcaatggtggggtgcccttcggttttctgctccgagtacgtaacagcgtcaccatcatggctacaaatgcaagtcctacgacaattaaaaaaagagcttccgtcgaaacacccgtcgaaccttcttccgatggaatctggactggtgcttgaagtgcctccatccgaggaaagggttccgatgcgtttagagttatcattatcgcgtctgcgttcgtagccgtctcgttccaaccatattcggaagtcggagtaggatctgatgactcccaaaccgaggtagcgttcaccgaagtatagttcgcaataggctccgctgtcgtaaccttctcgacaacacggtttaccggtgatgaaaccgttactttcaattttataacttcgaattgaaggaagaattccagatcataaacatcttcagcaaagaaagtcacgttaaactctttcttcattcgattcagatggaaaacacactgagaactcgttacacacgtatcccaataactcactagtctatgagtccccaccctgtcagtcagatgaacactcatcaaccaaaacggtgacctactcaaatctatctgtaacttgtgtccgaccgttacattcatatcaggtaatttactgacaatcataccggcggttgtattcttatcgaccaagcatcctgccgtcggcggaacgtttatatgggcacctccattggggtttaacattgtacggtattgcataatcggaaaatgctccttagtatacatacaatagtgagacgggcgtccgagaggatccggtgtgcgtgtacaatacatagtgcgaacagaacccccggtcataatttgtctatttgctaagggagcaacagaatcggatacctggtaaaatccctgaggcgtaatgacgtgaactaaatatatacgggcattcggatttaagtgatggatccacagagaaccttccgccaactcggtatacgctatctcggtggttacatcgtatttcccatatcttaaagtctgcacactatagcctcccatatatacgctgctatcatgtgaagcaactactataatcataatagaagaaacaaagtccttcttaaaatttggggaatacgacatttccgtcatatactttatgctgtaatggttgaagtaactgtcatatctataatcacgactaagtgtatacccattccaagtactccttaccggtcctaccctcgacccttcctgtaatacatggaacacaggcaaacctgtctttacatccagggttttcaaaaactttggaacaatcattcgatgatagcatccacttaaactaaacgtattaccccaggaaaattcctcacatactgtcgctccccaaacattttctccgcatactcttccggaccatccaccgtgtataccacagcttctaccgcccttatcttccaccattaaatcttccgaagccgtgtacccaccagtgatccacgaatactgagtctttagaacgaccacataatccgcatccaacttatctaatccaccgcttacaaatgtcggttctagcccgactattctgatacaccgatggcccttgctcatttgtgaatactgtctacatatcgtcgagcaagcatgagctcctgccgagtgacctatacagtgcaattttttagcgtcggggatatctaccagaaacttcctaaaatccgcatgtaaaccatccgtatcatagtacaaccgatagtccaccaacacaacacctacggcgggagtcatcttctgatgaaatcgcaacaccttcctaaaatcgtcatatcccagataccatcctggtataagcagcactatgtctgatttcccggcgaaggcattgtgcattttatggtatacaccatactcgtatctcgcatcgtggaacttcggtacaccaccatgcgatccataccacgtgattctcgaaggaagtctgttcggatttccggcgcttttcggagcttccagtttagtagccggaggcattgccacacaggaccgattgaccaaatcatggcaaccttctgatttcgtacccgaaaatgcggaggccccgaggagcaccccgaataactgaaacagaacgcaaaatttagaccggtaccctcccatacgattatcacgtcccaaagccaaatatcacggtactcaccagcgcaaaaatcttcatgaagatctggggcaagagccgcacaacagtccacctgaatctgagacagcttaccggcgactgtaccaaaccggtgtgccaccgccgaatttattctctcaatctattaatgtttaactaaacaaacttgctgacacttgataaatatttactgacctagacaattccgagaacttccttattaccgtgactatgcagtatcaagataaacccttccaaagttcgactgagtacacggtgtacttcctgtcataaaatatcacttctaaatatagtcctaggtagaaactataaatggtaagagacaacacactgattcttagaaaaacctcacagaacaagatgaacctcacattatcctgactcttccttacgaactgaaataaccggtaagtcataaaaatgattttccttttgacattgcgtacgcggaagcaaactagaaaaatcgaacttggaattttccaagtcgagttaactattaacttgatgacgtcaattggattaatcattaactcgaattagttaatgattaactagatctggttaatgattaactagtgacgtcactagttaatcattaagctttctatgcatatgcatgagagattcatgcatatgaatgagagtctcatccatattcataaacctcatccatattcatgagcctctcatgcatatgcatgtttttacatgcatatgcatggacctcattcatattcatcaattcgttaatgtataacgctatgactcactgtatatgtttacgttgcctagcaacgttaatgatttacctgctgacgtggcagctccgcctcccggtaaatcatttacctggactttgttctttatgtttattcaccatggcaacgctaccatatatggacatccgactccgcctccccagttatacattaacgatggcgtgataggcggagctctctcccattggctcttaatgacgtagtccgggttaaccataagccagaaccgcctatataggtagagcaggtagacccggaacaccattcccatacggacctccatagagtgcggacctctacgggctctccataccggtaaatattttattccatttaatccaatcaaataaatcaataatcaactcaatgctgtgattctgcctcaaattcaatggtgattttctttaataaaaagcccaccccccttggcacccccctgtacacccccctgtacaggcgaccaccccctatggacacccccctgtacaggcgaccaccccctatggacacccccctgtacaggcgaccaccccctatggacacccccctgtacaggcgaccaccccctatggacacccccctgtacaggcgaccaccccctatggacacccccctgtacacccccctgtacattttctcccataggctacaatggaacactgccccctagtgtctcccgctccatgggacccctatgaggtgggcaccatctcatttgccgcaatggagctcatccacgagggggcgccattgaagctaggggaccgcatagagagcctggccaatggggtgctttggaatccggatatccccgcccaactcttcaactgcatttctattcgctcatggggatcacatgggaagcgcgtcatattcaaaggccacacccaccggatgttccacgcccagcttaggatccgtagcaccgcccccgttactaggaaacaggccggaagcctactcctcagcctatcacagaggctcctgtgtttccccgcccgctataatacccaccccctcgtgatgcaattgggggtggagtctaatgccatgggacttcctatatattccaagagggccctcgagatggcgctcaagagcatgcgggtgcgcattgcgcctaacagccaccaggtggcgccacctgaaataggaaagacctgtacggtgaagcccctcaaagaagtggagaccctccagcagggggtcttcagtaccaccgatctaaaaagagcacttccagaatggacttttcgccgactttttaacgaaattccctatatttgtggctggaagattggcactgctccaaagggcggagaaatggatggttacgctccaccccgaatccagagccccgcccaccgaaggacggaaggacccgcccactctccaagacctcgcccggctgggcgtggtcgaaaactgcctcaagatgaggaggcggggcataagccctaggcaccacccctactttcaataaaccaatcagaacagagcacttgactcctcctatttgtgggcggggctatgggtacggtatagagcgccccctggcggccgttggccgccactgcacccgcgccggacttagtctctggcgcgggccggtcaatcattaacccggcgcccagcacgggcgccccctgccggccggagacagacactgcgtgtctgcggagctccccctggcggccgagggccgccactgcacccgcgccggacttagtctctggcgcgggccggtcaatcattaacccggcgcccagcacgggcgccccctgccggccggagacagacactgcgtgtctgcggagctccccctggcggccgagggccgccactgcacccgcgccggacttagtctctggcgcgggccggtcaatcattaacccggcgcccagcacgggcgccccctgccggccggagacagacactgcgtgtctgcggagctccccctggcggccgagggccgccactgcacccgcgccggacttagtctctggcgcgggccggtcaatcattaacccggcgcccagcacgggcgccccctgccggccggagacagacactgcgtgtctgcggagctccccctggcggccgagggccgccactgcacccgcgccggacttagtctctggcgcgggccggtcaatcattaacccggcgcccagcacgggcgccccctgccggccggagacagacactgcgtgtctgcggagctccccctggcggccgagggccgccactgcacccgcgccggacttagtctctggcgcgggccggtcaatcattaacccggcgcccagcacgggcgccccctgccggccggagacagacactgcgtgtctgcggagctccccctggcggccgagggccgccactgcacccgcgccggacttagtctctggcgcgggccggtcaatcattaacccggcgcccagcacgggcgccccctgccggccggagacagacactgcgtgtctgcggagctccccctggcggccgagggccgccactgcacccgcgccggacttagtctctggcgcgggccggtcaatcattaacccggcgcccagcacgggcgccccctgccggccggagacagacactgcgtgtctgcggagctccccctggcggccgagggccgccactgcacccgcgccggacttagtctctggcgcgggccggtcaatcattaacccggcgcccagcacgggcgccccctgccggccggagacagacactgcgtgtctgcggagctccccctggcggccgagggccgccactgcacccgcgccggacttagtctctggcgcgggccggtcaatcattaacccggcgcccagcacgggcgccccctgccggccggagacagacactgcgtgtctgcggagctccccctggcggccgagggccgccactgcacccgcgccggacttagtctctggcgcgggccggtcaatcattaacccggcgcccagcacgggcgccccctgccggccggagacagacactgcgtgtctgcggagctccccctggcggccgagggccgccactgcacccgcgccggacttagtctctggcgcgggccggtcaatcattaacccggcgcccagcacgggcgccccctgccggccggagacagacactgcgtgtctgcggagctccccctggcggccgagggccgccactgcacccgcgccggacttagtctctggcgcgggccggtcaatcattaacccggcgcccagcacgggcgccccctgccggccggagacagacactgcgtgtctgcggagctccccctggcggccgagggccgccactgcacccgcgccggacttagtctctgacaccgcatttactttcaacacctttttttatttcagcacaccgaaatctcgtccgtgtaaaccttgtccccaaacctcagtcccgtacatcgaacccatccacatatatctcgcacagctccagtgcttacaagatatttccctactggataattaggatcttgacaccacttattcaaatacatccggaaccactgtccgtctggaacttggcttctgtagaactcctcacgaaagtagcgcttcattgctctagaacacttatacaaatgtttatctctcaggtcgaacatcgtgaggcaaatcaacagcgtcaaatgacaagcacaagaaccgcccggctgaagcccgacgcagtaacccataggatgtccgacaccgatgttagcttcttcgtggtacggataccacagctccttgatgtcttgaactagcttccagaagatggcatcgtgcatacaccacggaggtacggcaacaccaaacaccacgtacaaaggcatctcccgacactctgcaattacaactagcatcagaaatacatccagccgctatttgaaaaaaacaacaggatctcacccaaaaagaaaaagtacttaccccgaaaccaccaggaaatcccccttacgtgataatccggatctcgctgacgctcaaagaagccgccttaaataccgctccttatctctcttcgattacctcagttacgcccatttcttatcaggtaagatacgcaggtaagatacgcccttccacatcagcacggaatgtgctgaccagcttaccgcgcccgtttttaatatccgttaattagtaacttaggtgaatcaccaaaccacctgccggcatatatctacacccttgatacggcggcatccattgaagtcgagcgccaccatggagtcaactaccgtatcctcgattctgctcctatccttcttcgtatcttccatcgaatcctatccgctcctgcataacttcacggcgctcacgggatccgtgcttactcttccctacaaaggacatgaccgaccctttaaattcgaatggcggctgacagatcagaccaaagtagcaatctcggatcctagcaccggcatcaactacccgtcgggtccactcaaaggaagagtacatctaaacggcagcgccctcatcgttacatccctacgacttagtgacgccggtacctatacaatcctctcagaggacaacacaggaactgaaatcggatactcctattacgtcgaagtcagaggtatagaactttcccctcctttttctacatgatatcccgttccctcttttttcttacccctagcttattcttcctagaaccgatgcaagctcccaccctctatacggatcgctacaatgactcatctgccatacgcctcacatgccaagcttccaacaatctccaccgtaatatcacataccactggaaaacagatttaatacagccaactaactcgactcgatctatcaccttaaacatcgaagactatatatccgttacctgcacagtcactgatggagtcagcaaaaacagcatcacgattatggttccgttgagaggtagtattcggtttcccgttatctccctatactacgtaatcatgcccacccttttaacccgtatctttacaacagatccttctccacctacgccttacggtttgcatcccactatcattttcctgagtgtcctctgcatgatcctcatcaccgcaattaccgtctactttgtgaagaagcattgctgcgataagcaatataaaataacttgcattaacccttaccgagaatgcttcggtggcgccggtctcgtttaatctcgtttaaataaaaaccactataatccccgcttcctataatctctacttcctatgattaaatgggtaattaaatgatgggtaattaagtggtgtcaatgatcaaataatgattcggaaacgatttcgggaaaaatgattttaggaatcaatgatcattatcaaaaataaatgatttatttataagacgtgtttttgatgattgatacgattagtaaatcacatgattagaaacacatgattagaaacacagtttaatcatcaatcgaaatcaccgcgcaagatatggacagtcacgttctcctctgatgtcctatccatagattcgctgtccgtagaatcagaggcgcagagcatccgccgaaaccagaaagttatcgctaccatcagcaataacaacataattaacgcgatcggcagccacactggaaactcgccggtctgattggataccagtcctccgccggtcttataagtggtctcctcgatcttctgatcctcctgagtcaaaccaggaattaccactacgtaaaatccggtctttgaatcctgttgtaagtctagcgtattagtatacagtcccgaatcggcaggtgttacgtctctaatagtaacgcaattggatgtggcattgtaatgcgtgcggctcttatagttagcatacactatggggttacccagagctttataaagctgtaatacgaacacggtagacgcgtgctcgttagaggactgaaactcccactccgttatagaagcggagctagcatccttcccacacatgcgtaactctccaccttccaaaactaatatacggctcatgttatgcacctcaaccgtcgcattgcccgtaatatccttcacggtatactgtatggcatacggtttcccaccgacaaaggaaccgtaagtcaaccagcacccgttattagccttcagcttactcaggtaaatagtattgcaaccactatctaccctcgttctacccatgtacccgctttcaagtccaggttctttaaccctcggaatcacaaatgccgccctctccatcttattgcaattgggggacggggaatgataccagaggatcatagtatggtccctgcactctcctgtccgtagagccagctccgggtcccggggagcgccaaagcagagtccgaggacagcagccagcagcagggcaacggacttcatgatgaatgcgggaaccagccagcagcagcaggtagaaggtgcgagtactcgaggcaggcgggaataacaccgcacgctttccaccccgcttaaatacacaacccacaccggtcatggtcaaacattacctagcctactcagcacggaaaagtactcacccttaacacagttcgacttatcaggtacacacccgtaaccttcgcaccccaaagcgcacagtcagcaccataaggaagtcgtaaagttaccctttgattgcattgtcatcataaaaaacgctgagcaaacggaaacgccccaagtacaaatctctcttccgccacgccctcgttaatcaataactagtcgccgatacatatataccccctccgttccatcacacctacactaccttctctccgcacaggcaacatctcaatccttactcttccgaatccacttcgccgccttcgacatgaatccggtaagtatcaacttttttctaagcttatgcttctgacacctctgatcttaataccgcaccccttttttctcaaaaaaggtttcgtgcttaacgcttcttctatgcgtcatcatcccgagagccgatccgcttccaatcacccccgcctctaaacccgctaccgactccgcccggaccggcgcctccgtcatcacgacccacttacccgcatctccgagcgccaccccgtgcgacgaaatcttgagcgaggactgttggttcgaaaatgccagcggtgattaccaacccctaccctgggaaccgaaagaggaaacggtttcagatcaaaaccctctcaccgcaaccgaccccatcggtgaccgaatccccgctatcatccagtcccagtcccgcgcttctaaccgtccgaccagtaaggaacacacttctactatcgcatccatctcgaccgtagtcggcatcgcggtcctcgtcatcctgaccctcgtagcctactttaccaagtaccccaaaccgagaccgcccagatccatctacataggagtagctccacccgatatggaactcaaggaaatataattccagccccacccttaaccctacctttccatgagtcagtattttcaataaagttatattgcagtattaattccgttgtttccgcgttctttctctcgcgcggacaaagtccgttcgaccaggaagtccggtatacgtcattccgcggtgtcatgatgacgcgcataactcacgactgccatctgccggacaaacgcggtactacacttaacacataaacacccgccttttttcgattcccaccataatcaggctttggtaaaaattcgcagattctaaaatccgtattcctgcgcccgcgataatagatcacgcccacgacacgccctagcgctcttatcacacggtctctgctgccatctagcgggcgggagcggtagtgcgaggtgacagcagcgtcattcatgtaggtatatatagatgatg

SEQ ID NO: 2 - DNA, 714 bp, Aequorea  victoria
  gene (1)..(714): Enhanced green fluorescent protein (EGFP)
gtgagcaagggcgaggagctgttcaccggggtggtgcccatcctggtcgagctggacggcgacgtaaacggccacaagttcagcgtgtccggcgagggcgagggcgatgccacctacggcaagctgaccctgaagttcatctgcaccaccggcaagctgcccgtgccctggcccaccctcgtgaccaccctgacctacggcgtgcagtgcttcagccgctaccccgaccacatgaagcagcacgacttcttcaagtccgccatgcccgaaggctacgtccaggagcgcaccatcttcttcaaggacgacggcaactacaagacccgcgccgaggtgaagttcgagggcgacaccctggtgaaccgcatcgagctgaagggcatcgacttcaaggaggacggcaacatcctggggcacaagctggagtacaactacaacagccacaacgtctatatcatggccgacaagcagaagaacggcatcaaggtgaacttcaagatccgccacaacatcgaggacggcagcgtgcagctcgccgaccactaccagcagaacacccccatcggcgacggccccgtgctgctgcccgacaaccactacctgagcacccagtccgccctgagcaaagaccccaacgagaagcgcgatcacatggtcctgctggagttcgtgaccgccgccgggatcactctcggcatggacgagctgtacaag

SEQ ID NO: 3 - DNA, 711 bp, Discosoma  sp
  gene (1)..(711): mCherry Red protein
atggtgagcaagggcgaggaggataacatggccatcatcaaggagttcatgcgcttcaaggtgcacatggagggctccgtgaacggccacgagttcgagatcgagggcgagggcgagggccgcccctacgagggcacccagaccgccaagctgaaggtgaccaagggtggccccctgcccttcgcctgggacatcctgtcccctcagttcatgtacggctccaaggcctacgtgaagcaccccgccgacatccccgactacttgaagctgtccttccccgagggcttcaagtgggagcgcgtgatgaacttcgaggacggcggcgtggtgaccgtgacccaggactcctccctgcaggacggcgagttcatctacaaggtgaagctgcgcggcaccaacttcccctccgacggccccgtaatgcagaagaagaccatgggctgggaggcctcctccgagcggatgtaccccgaggacggcgccctgaagggcgagatcaagcagaggctgaagctgaaggacggcggccactacgacgctgaggtcaagaccacctacaaggccaagaagcccgtgcagctgcccggcgcctacaacgtcaacatcaagttggacatcacctcccacaacgaggactacaccatcgtggaacagtacgaacgcgccgagggccgccactccaccggcggcatggacgagctgtacaagtag

SEQ ID NO: 4 - DNA, 553 bp, Human cytomegalovirus
  promoter (1)..(553): Immeadiate early promoter
atagtaatcaattacggggtcattagttcatagcccatatatggagttccgcgttacataacttacggtaaatggcccgcctggctgaccgcccaacgacccccgcccattgacgtcaataatgacgtatgttcccatagtaacgccaatagggactttccattgacgtcaatgggtggagtatttacggtaaactgcccacttggcagtacatcaagtgtatcatatgccaagtacgccccctattgacgtcaatgacggtaaatggcccgcctggcattatgcccagtacatgaccttatgggactttcctacttggcagtacatctacgtattagtcatcgctattaccatggtgatgcggttttggcagtacatcaatgggcgtggatagcggtttgactcacggggatttccaagtctccaccccattgacgtcaatgggagtttgttttggcaccaaaatcaacgggactttccaaaatgtcgtaacaactccgccccattgacgcaaatgggcggtaggcgtgtacggtgggaggtctatataagc

SEQ ID NO: 5 - DNA, 584 bp, Cytomegalovirus
  enhancer (1)..(584): CMV enhancer/ chicken beta-actin promoter (CAG)
gcgttacataacttacggtaaatggcccgcctggctgaccgcccaacgacccccgcccattgacgtcaataatgacgtatgttcccatagtaacgccaatagggactttccattgacgtcaatgggtggagtatttacggtaaactgcccacttggcagtacatcaagtgtatcatatgccaagtacgccccctattgacgtcaatgacggtaaatggcccgcctggcattatgcccagtacatgaccttatgggactttcctacttggcagtacatctacgtattagtcatcgctattaccatggtcgaggtgagccccacgttctgcttcactctccccatctcccccccctccccacccccaattttgtatttatttattttttaattattttgtgcagcgatgggggcggggggggggggggggcgcgcgccaggcggggcggggcggggcgaggggcggggcggggcgaggcggagaggtgcggcggcagccaatcagagcggcgcgctccgaaagtttccttttatggcgaggcggcggcggcggcggccctataaaaagcgaagcgcgcggcgggcg

SEQ ID NO: 6 - DNA, 1190 bp, Homo sapiens
  promoter (1)..(1190): Human elongation factor 1 alpha (EF1A) promoter
cgtgaggctccggtgcccgtcagtgggcagagcgcacatcgcccacagtccccgagaagttggggggaggggtcggcaattgaaccggtgcctagagaaggtggcgcggggtaaactgggaaagtgatgtcgtgtactggctccgcctttttcccgagggtgggggagaaccgtatataagtgcagtagtcgccgtgaacgttctttttcgcaacgggtttgccgccagaacacaggtaagtgccgtgtgtggttcccgcgggcctggcctctttacgggttatggcccttgcgtgccttgaattacttccacgcccctggctgcagtacgtgattcttgatcccgagcttcgggttggaagtgggtgggagagttcgaggccttgcgcttaaggagccccttcgcctcgtgcttgagttgaggcctggcctgggcgctggggccgccgcgtgcgaatctggtggcaccttcgcgcctgtctcgctgctttcgataagtctctagccatttaaaatttttgatgacctgctgcgacgctttttttctggcaagatagtcttgtaaatgcgggccaagatctgcacactggtatttcggtttttggggccgcgggcggcgacggggcccgtgcgtcccagcgcacatgttcggcgaggcggggcctgcgagcgcggccaccgagaatcggacgggggtagtctcaagctggccggcctgctctggtgcctggcctcgcgccgccgtgtatcgccccgccctgggcggcaacaggctggcccggtcggcaccagttgcgtgagcggaaagatggccgcttcccggccctgctgcagggagctcaaaatggaggacgcggcgctcgggagagcgggcgggtgagtcacccacacaaaggaaaagggcctttccgtcctcagccgtcgcttcatgtgactccacggagtaccgggcgccgtccaggcacctcgattagttctcgagcttttggagtacgtcgtctttaggttggggggaggggttttatgcgatggagtttccccacactgagtgggtggagactgaagttaggccagcttggcacttgatgtaattctccttggaatttgccctttttgagtttggatcttggttcattctcaagcctcagacagtggttcaaagtttttttcttccatttcaggtgtcgtga

SEQ ID NO: 7 - DNA, 114 bp, Fowlpox virus
  misc_feature (1)..(114): Promoter Sequence for L2R (Fowlpox promoter)
catagtaaatatgggtaacttcttaatagccataattaaaattgaaaaaaaaatatcattataaaacgtaaacgaacaaaaaacattaatttaaatttgccaataacaaaccat

SEQ ID NO: 8 - DNA, 276 bp, eukaryotic cells
  misc_feature (1)..(276): Promoter Sequence for B-actin (minimal)
tcgaggtgagccccacgttctgcttcactctccccatctcccccccctccccacccccaattttgtatttatttattttttaattattttgtgcagcgatgggggcggggggggggggggcgcgcgccaggcggggcggggcggggcgaggggcggggcggggcgaggcggagaggtgcggcggcagccaatcagagcggcgcgctccgaaagtttccttttatggcgaggcggcggcggcggcggccctataaaaagcgaagcgcgcggcgggcg

SEQ ID NO: 9 - DNA, 516 bp, Woodchuck hepatitis virus
  misc_feature (1)..(516): Woodchuck hepatitis virus post-transcriptional regulatory element (WPRE)
tcaacctctggattacaaaatttgtgaaagattgactggtattcttaactatgttgctccttttacgctatgtggatacgctgctttaatgcctttgtatcatgctattgcttcccgtatggctttcattttctcctccttgtataaatcctggttgctgtctctttatgaggagttgtggcccgttgtcaggcaacgtggcgtggtgtgcactgtgtttgctgacgcaacccccactggttggggcattgccaccacctgtcagctcctttccgggactttcgctttccccctccctattgccacggcggaactcatcgccgcctgccttgcccgctgctggacaggggctcggctgttgggcactgacaattccgtggtgttgtcggggaagctgacgtcctttccatggctgctcgcctgtgttgccacctggattctgcgcgggacgtccttctgctacgtcccttcggccctcaatccagcggaccttccttcccgcggcctgctgccggc

SEQ ID NO: 10 - DNA, 1695 bp, Influenza A virus (A/chicken/Mexico/435/2005 (H5N2))
  gene (1)..(1695): Segment 4 Hemagglutinin gene
atggaaagaatagtgattgcctttgcaataatcagcattgttacaggtgaccaaatctgcattggttatcatgcaaacaattcaacaaaacaagttgatacaatcatggaaaagaatgtgacggtcacacatgctcaggacatactagaaaaagaacacaatggaagactctgcagtcttaaaggagtaaagcccctcatcctgaaggattgcagcgtagctgggtggattctgggaaatcctatgtgtggtgaattcctgaatgtgccggaatggtcatacattgtggagaaagacaacccatccaatggcctgtgttaccctggaaacttcgacaattatgaagaattgaagcatttaatgagcagcacaaatcacatcgagagaattcagatatttcctaggagctcttggtccaaccataatgcctcatcaggagtgagctcggcatgcccgtccaatggtatatcttcctttttccggaatgtagtgtggttgatcaagaaggataatgtgtaccgaacactaaagaagaactacaccaacaccaatgtagaagaccttttaataatgtggggagttcatcaccctactgatgcaactgagcagacaaaactctaccagaacctgaacacttatgtatcggtgggaacatcaacactaaatcagaggtcaatcccgaaaatagccaccagaccccaggtgaacggacagagaggaaggatggaatttttttggacaatattaaagccgaacgattcaatcttttttgagagtactgggaactttatagctcccgaatatgcatacaagatcactaaaaaagggaaatcagcagtcatgaaaagtgaactggattatggcgactgtaataccaaatgccagaccccagtgggtgctgtaaattccagtctgcctttccacaatgtccatccctttaccattggggaatgccccaggtatgtaaaatcgaagaaactggtccttgcaacaggattaagaaatgtaccccaaaaagaaacaagaggcttatttggagcaatagctggattcatagaaggggggtggcaaggaatggtggatggatggtatggataccatcatagcaatgagcagggtagtgggtatgctgcagacaaagaatctacacagaaagcaattaatggaatcactaataaagtcaactcaatcattggcaaaatgaacactcagttcgaagccattgggaaagaattcaacaacctagaaaggagaatagaaaatttgaataagaaaatggaagatgactttttggatgtatggacttacaatgcagaacttctagtgctcatggaaaacgagagaactctggatctccatgattcaaatgtcaagaatttatacgataaggtccgactccaactgagagataatgcaaaagaactaggcaacggatgctttgaattctaccacaagtgtgacaatgaatgcatggaaagtgtgagaaatggaacgtatgattacccacaatactcaaaagagtcaaaactgaatagagaggaaatagaaggggtcaaattagaatcaacagggacttatcagatactttcaatctattcaacagtggcgagttccctagcactggcaatcatggtagctggtctatctttttggatgtgctccaatggatcattgcagtgcagaatttgcatctaa

SEQ ID NO: 11 - DNA, 1723 bp, Influenza A virus (A/chicken/Jalisco/CPA1/2012(H7N3))
  gene (1)..(1722): Segment 4 Hemagglutinin gene
ggatacaaaatgaacactcaaattttggcactcattgcttgtatgctgattggagctaaaggagataaaatatgtcttgggcaccatgctgtggcaaatggaacaaaagtgaacacattaacagagagaggaatcgaagtagtaaatgccacagaaacggtggagactgcaaatactaagaaaatatgcactcaggggaaaagaccaacagatctgggacaatgcggacttctaggaaccctaataggacctccccaatgcgatcaatttctggaatttgacgctgatttaataattgaacgaagagaaggaaccgatgtgtgttatcccgggaagttcacaaatgaagaatcactgaggcaaatccttcgagggtcaggaggaattgataaagagtcaatgggtttcacctatagtggaataagaaccaatggggcgacaagtgcttgcagaagatcaggttcttccttctatgcggagatgaagtggttactgtcgaattcagacaatgcggcttttccccaaatgactaagtcgtacagaaatcccaggaacaaaccagctctgataatttggggagtgcatcattctggatcggctactgagcagaccaaactctatgggagtggaaacaagttgataacagtaggaagctcgaaataccagcagtcattcaccccaagcccgggggcacgaccacaggtgaatgggcaatcaggaaggattgattttcactggctactccttgaccccaatgacacagtgaccttcactttcaatggggcattcatagcccctgacagagcaagtttctttagaggagagtcaataggagttcagagtgatgttcctttggattctggttgtgagggggattgcttccacaatgggggtacgatagtgagttccctgccattccagaacatcaaccctagaacagtgggaaaatgccctcgatatgtcaaacagacaagcctccttttggctacagggatgagaaacgtcccagagaaccccaaggataggaagagccgacatcgaaggaccagaggcctttttggagcgattgctggattcatagagaatggatgggaaggtctcattgatggatggtatggtttcagacatcaaaatgcacaaggagaaggaactgcagctgattacaaaagcactcaatctgcaatagatcagatcacaggcaaattgaatcgtctaattgacaaaacaaatcagcagtttgaactgatagacaacgaattcagtgaaatagaacaacaaattgggaatgtcattaactggacacgagattcaatgactgaggtatggtcgtacaatgctgaattgctggtagctatggaaaatcagcacacaatagatcttgcagactcagaaatgaacaaactttatgagcgtgtaaggaaacaactgagggagaatgctgaagaggatgggactggatgctttgagatatttcataagtgtgatgatcagtgcatggagagcatcaggaacaacacttatgaccatactcaatacagagcggagtcattgcagaatagaatacagatagacccagtgaaattgagtagtggatacaaagacataatcttatggtttagcttcggggcatcatgttttcttcttctagccattgcaatgggattggttttcatttgcataaagaatggaaacatgcggtgcactatttgtatatagtttgaga

SEQ ID NO: 12 - DNA, 1723 bp, Influenza A virus (A/chicken/Guanajuato/07437-15/2015(H7N3))
  gene (1)..(1722): Segment 4 Hemagglutinin gene
ggatacaaaatgaacactcaaattttggcactcattgcttatatgctaattggagctaaaggagacaaaatatgtcttgggcaccatgctgtggcaaatggaacaaaagtgaacacattaacagagaggggaatcgaagtagtaaatgccacagaaacggtggagactgcaaatactaagaaaatatgcactcaggggaaaagaccaatagatctaagacaatgcggacttctaggaaccctaataggacctccccaatgcgatcaatttctgaaatttgacgctgatttaataattgaacgaagagaaggaaccgatgtgtgttatcccgggaagttcacaaatgaagaatcactgaggcaaatacttcgaagatcaggaggaattgataaagagtcgatggatttcacctataatggaataagaaccaatgggacgacaagtgcttgcaaaagatccaatccttccttctatgcggagatgaagtggttactgtcggattctgacaatgcaactttccctcaaatgactatgtcgtacagaaatcccaggaacaaatcagctctgataatttggggagtgcatcattctggatcggctactgagcagaccaaactctatgggagtggagacaagttcataacagtaggaagctcgaaatacctgcagtcattcaccccaagcccggggccacgaccaaaggtgaatgggcaatcaggaaggatcgactttcactggctactccttgatcccaatgacacagtgaccttcactttcaatggggcattcatagctcctgacagagcaagcttctttagaggagagtcaataggaattcagagtgatgttcctttggatcctggttgtaagggggattgcttccacaatgggggtacgatagtgagttctctgccattccagaacatcaaccctagaacagtgggaaaatgccctcggtatgtcaaacagccaagcctccttttggctacagggatgagaaatgtcccagagaaccccaaggataggaagagccgacatcgaaggaccagaggcctttttggagcgattgctgggttcatagagaatggatgggaaggtctcattgatggatggtatggtttcagacatcaaaatgcacaaggagaaggaactgcagctgattacaaaagcactcaatctgcgataaatcaaatcacaggcaaattgaatcgtctaattgacaaaacaaatcagcagtttgaactgatagacaacgaattcagtgaaatagaacaacagattgggaatgtcattaactggacacgcgattcaatgactgaggtatggtcgtacaatgctgaattgctgatagctatggaaaatcagcacacaatagatcttgcagactcagaaatgaacaaactttatgagcgtgtaaggaaacaacttagggagaatgctgaagaggatgggactggatgctttgaaatgtttcataagtgtgatgatcagtgcatggagagcatcaggaacaacacttatgaccatactcaatacagagcggaatcattgcagaataggatacagatagatccagtgaaattgagtagtggatacaaagacataatcttatggtttagcttcggggcatcatgttttcttcttctagccattgcaatgggattggttttcatttgcataaagaatggaaacatgcggtgcactatttgtatatagtttgaga

SEQ ID NO: 13 - DNA, 2652 bp, Gallid herpesvirus 1 strain USDA
  gene (1)..(2652): Laryngotracheitis virus (ILT) glycoprotein B
atgcaatcctacatcgccgtgaacattgacatggctagcttgaaaatgctgatctgcgtgtgcgtggcaatcctgatcccatctaccctatctcaagattcacacggaattgctggaataatagaccctcgtgatacagccagcatggatgttggaaaaatctctttctccgaagccattgggtcgggggcaccgaaagaaccccagattagaaacagaatttttgcgtgctcatctccaactggcgccagtgttgcgaggcttgcccagccacgacattgtcaccgacatgccgattcgactaacatgactgaaggaattgccgtagtcttcaagcaaaacattgccccgtacgtctttaatgtgactctatactataaacatataaccacagttactacgtgggcattattctcaagaccccaaataacaaatgagtacgtgaccagggttccaatagactatcatgaaattgtcaggattgatcgatcgggagaatgctcatccaaagcaacgtatcataaaaatttcatgttttttgaagcttacgacaatgatgaagcagaaaaaaaattgcccctggttccatcactgttaagatcaactgtctccaaggcgtttcatacaactaactttactaagcgacatcaaaccctgggataccgaacgtctacatcggtcgactgtgttgtgaaatatctacaggctagatctgtatacccgtatgattactttggaatggcgacaggtgatacagtagaaatttctcctttttataccaaaaacacgaccggaccaaggcgtcacagtgtctacagagactatagatttctcgaaatcgcaaattatcaagtcagggatttggaaaccggacaaataagaccccctaaaaaaagaaactttctaacagatgaacaattcactataggctgggatgcaatggaagaaaaggaatctgtatgtactctcagtaaatggattgaagtcccggaagcagttcgtgtttcgtacaaaaacagttaccacttttcacttaaagatatgactatgacgttctcgtccggaaaacaaccttttaacatcagcaggcttcatttggctgaatgcgttcctaccatagcctcggaggccatagatggcatctttgccagaaagtatagttcgactcatgtccgttctggggacatcgaatactatctcggtagtggcggatttctgatcgcatttcagaaactcatgagccatggcttggctgaaatgtacctagaagaggcacaaagacaaaatcatctcccgagagggagagagcgtcgccaagccgcaggtcgccgcacggcgtcgctgcagtctggacctcagggtgatagaattactacccacagttctgcaacatttgccatgttacaatttgcatacgacaaaatccaagcccatgttaacgagcttatcggaaatttgttggaagcgtggtgtgagcttcagaaccgccaactgattgtatggcatgagatgaagaaactaaacccgaactcactgatgacatctttgttcggacaacctgtaagcgccaggctattgggagacatcgtagcggtatcaaaatgtatagaaattccaatcgaaaatattaggatgcaggattccatgcgcatgccaggggacccaaccatgtgctataccagaccagtacttattttcaggtattcgtcctcccctgagtcacagttttctgcgaactcaacagaaaaccacaatcttgacatattaggccaactcggagaacataatgaaattttacaagggcggaatttgatagaaccatgcatgatcaatcacagacggtactttctgttgggagaaaactaccttctttacgaagactatacatttgttagacaagtaaatgcttccgagatcgaagaagtgagcacattcatcaacttgaacgccactatactagaagatttggactttgtgcccgtcgaagtatacactcgcgaggaactcagagatactgggactttaaactatgatgatgtggtcagatatcaaaatatttataacaaaaggttcagagacattgacactgtaatacgtggagataggggagatgcaatctttagagcaatagcagatttttttggcaacactcttggagaagtaggaaaggcattgggaactgtagtgatgacagccgcggcagcagtaatttctacagtatctggcatcgcctcatttctttctaacccgttcgccgcactcggaattgggatagcggtggtggtgagcattattttaggactgctggcgttcaaatatgtaatgaacctgaaatcaaacccagttcaggttctgttcccaggcgcagttcccccggccggaactcctccacgaccctctagacgttactacaaggatgaggaggaggttgaggaggatagtgatgaggacgacaggatacttgccaccagagttctgaaaggccttgagcttctacacaaggatgaacagaaagctcgaagacagaaagcgcggttttctgcttttgctaaaaatatgagaaacctatttcgcagaaaaccccgaaccaaggaagatgactaccccctgctcgaatacccttcgtgggcagaagaaagcgaagacgaataa

SEQ ID NO: 14 - DNA, 1305 bp, Gallid herpesvirus 1 strain USDA
  gene (1)..(1305): Laryngotracheitis virus (ILT) glycoprotein D
atgcaccgtcctcatctcagacggcactcgcgttactacgcgaaaggagaggtgcttaacaaacacatggattgcggtggaaaacggtgctgctcaggcgcagctgtattcactcttttctggacttgtgtcaggattatgcgggagcatatctgctttgtacgcaacgctatggaccgccatttatttttgaggaatgctttttggactatcgtactgctttcttccttcgctagccagagcaccgccgccgtcacgtacgactacattttaggccgtcgcgcgctcgacgcgctaaccataccggcggttggcccgtataacagatacctcactagggtatcaagaggctgcgacgttgtcgagctcaacccgatttctaacgtggacgacatgatatcggcggccaaagaaaaagagaaggggggccctttcgaggcctccgtcgtctggttctacgtgattaagggcgacgacggcgaggacaagtactgtccaatctatagaaaagagtacagggaatgtggcgacgtacaactgctatctgaatgcgccgttcaatctgcacagatgtgggcagtggactatgttcctagcacccttgtatcgcgaaatggcgcgggactgactatattctcccccactgctgcgctctctggccaatacttgctgaccctgaaaatcgggagatttgcgcaaacagctctcgtaactctagaagttaacgatcgctgtttaaagatcgggtcgcagcttaactttttaccgtcgaaatgctggacaacagaacagtatcagactggatttcaaggcgaacacctttatccgatcgcagacaccaatacacgacacgcggacgacgtatatcggggatacgaagatattctgcagcgctggaataatttgctgaggaaaaagaatcctagcgcgccagaccctcgtccagatagcgtcccgcaagaaattcccgctgtaaccaagaaagcggaagggcgcaccccggacgcagaaagcagcgaaaagaaggcccctccagaagactcggaggacgacatgcaggcagaggcttctggagaaaatcctgccgccctccccgaagacgacgaagtccccgaggacaccgagcacgatgatccaaactcggatcctgactattacaatgacatgcccgccgtgatcccggtggaggagactactaaaagttctaatgccgtctccatgcccatattcgcggcgttcgtagcctgcgcggtcgcgctcgtggggctactggtttggagcatcgtaaaatgcgcgcgtagctaa

SEQ ID NO: 15 - DNA, 1734 bp, Newcastle disease virus strain La Sota C5
  gene (1)..(1734): HN gene
atggaccgcgccgttagccaagttgcgttagagaatgatgaaagagaggcaaaaaatacatggcgcttgatattccggattgcaatcttattcttaacagtagtgaccttggctatatctgtagcctcccttttatatagcatgggggctagcacacctagcgatcttgtaggcataccgactaggatttccagggcagaagaaaagattacatctacacttggttccaatcaagatgtagtagataggatatataagcaagtggcccttgagtctccgttggcattgttaaatactgagaccacaattatgaacgcaataacatctctctcttatcagattaatggagctgcaaacaacagtgggtggggggcacctatccatgacccagattatataggggggataggcaaagaactcattgtagatgatgctagtgatgtcacatcattctatccctctgcatttcaagaacatctgaattttatcccggcgcctactacaggatcaggttgcactcgaataccctcatttgacatgagtgctacccattactgctacacccataatgtaatattgtctggatgcagagatcactcacattcatatcagtatttagcacttggtgtgctccggacatctgcaacagggagggtattcttttctactctgcgttccatcaacctggacgacacccaaaatcggaagtcttgcagtgtgagtgcaactcccctgggttgtgatatgctgtgctcgaaagtcacggagacagaggaagaagattataactcagctgtccctacgcggatggtacatgggaggttagggttcgacggccagtaccacgaaaaggacctagatgtcacaacattattcggggactgggtggccaactacccaggagtagggggtggatcttttattgacagccgcgtatggttctcagtctacggagggttaaaacccaattcacccagtgacactgtacaggaagggaaatatgtgatatacaagcgatacaatgacacatgcccagatgagcaagactaccagattcgaatggccaagtcttcgtataagcctggacggtttggtgggaaacgcatacagcaggctatcttatctatcaaggtgtcaacatccttaggcgaagacccggtactgactgtaccgcccaacacagtcacactcatgggggccgaaggcagaattctcacagtagggacatctcatttcttgtatcaacgagggtcatcatacttctctcccgcgttattatatcctatgacagtcagcaacaaaacagccactcttcatagtccttatacattcaatgccttcactcggccaggtagtatcccttgccaggcttcagcaagatgccccaactcgtgtgttactggagtctatacagatccatatcccctaatcttctatagaaaccacaccttgcgaggggtattcgggacaatgcttgatggtgtacaagcaagacttaaccctgcgtctgcagtattcgatagcacatcccgcagtcgcattactcgagtgagttcaagcagtaccaaagcagcatacacaacatcaacttgttttaaagtggtcaagactaataagacctattgtctcagcattgctgaaatatctaatactctcttcggagaattcagaatcgtcccgttactagttgagatcctcaaagatgacggggttagagaagccaggtctggctag

SEQ ID NO: 16 - DNA, 1716 bp, Newcastle disease virus strain M08-3313/Mexico
  gene (1)..(1716): Hemagglutinin neuramidase of Newcastle disease virus strain M08-3313/Mexico
atggatcgtgtagttagcagagttgtactagagaacgaagaaagagaagcaaagaacacatggcgcttggttttccggatcgcagtcttatctctaatagtaatgactttagctatctctgtagccgccctggtatacagcatgggggctagcacaccgagcgaccttgcaggcatatcaacggtgatctctaaggcagaggatagggttacatctttactcagttcaaatcaagatgtggtagatagggtatataaacaggtggcccttgagtccccgctggcgttgctaaatactgaatctataattatgaatgcaataacttctctctcttatcaaattaatggggctgcaaataatagtgggtgtggggcacctgttcatgacccagattatattgggggggtaggcaaagaactcatagtagatgacacaagtgatgtcacatcattctatccttcagcataccaagaacacctgaattttatcccggcgcctactacaggatcaggctgcactcggataccctcattcgacatgagcgctacccactattgttatactcacaatgtgatattatctggttgcagagatcactcgcactcacatcagtatttagcgctaggtgtacttcggacatctgcaacagggagggtattcttttctactctgcgttccatcaatttagatgacacccaaaatcggaagtcttgcagtgtgagtgcgactcctttaggttgtgatatgctgtgctctaaagtcatagagactgaggaggaggattataagtcaattacccccacatcaatggtgcatggaaggttagggtttgacggtcagcaccatgagaaggacttagacgtcacagtcttatttaaggattgggttgcaaattacccgggagtgggaggagggtctcttattgacgaccgtgtatggttcccagtttatggagggctaaaacccaattcgcctagcgacactgcacaagaagggagatatgtaatatacaagcgctataataacacatgccccgatggacaagattaccaagttcggatggctaagtcttcgtataagcctggacggtttggtagaaagcgcgtacagcaagccatcttatctatcaaagtatcaacatccttgggcgaggacccggtgctgactgtaccgccaaatacagttacactcatgggggctgaaggcagagtcctcacagtagggacatctcatttcttgtaccaacgagggtcttcatacttctctcccgccttattataccctatgacagtacacaacaaaacagctactcttcatagtccttatatatttaatgctttcactcggccaggtagtgtcccttgccaggcatcagcaaggtgccctaactcatgtatcactggagtctatactgatccgtatcctgtagtcttccataggaatcacaccttgcgaggggtgttcgggacaatgcttgataatgaacaagcaaggttcaaccccgtatctgcagtatttgattacacatctcgcagtcgcataacccgggtaagttcaagcagcaccaaggcagcatacacgacatcgacatgttttaaagttgtcaagaccaataaagtttattgccttagcattgcagaaatatccaacaccctatttggggaattcaggattgtccctttactggtcgagatcctcaaggatgatagggtttaa

SEQ ID NO: 17 - DNA, 1350 bp, Chicken anemia virus isolate CAV-10
  gene (1)..(1350): VP1 gene of Chicken anemia virus isolate CAV-10
atggcaagacgagctcgcagaccgagaggcagattttacgccttcagaagaggacggtggcaccacctcaagcgacttcgacgaagatataaatttcgacatcggaggagacagcggtatcgtagacgagcttttaggaaggcctttcacaacccccgccccggtacgtatagtgtgaggctaccgaacccccagtcaacgatgactatccgctttcaaggcatcatttttcttaccgaaggactcattctacctaaaaacagtacagcggggggatatgcagaccacctctacggggcgagagtcgccaagatctcagtgaacctgaaagagttcctgctagcgtcaatgaacctgacatacgtgagcaaaataggaggccccatcgccggtgagttgattgcggacgggtctcaatcacaagccgcgcaaaactggcctaattgctggctgccgctagataataacgtgccctccgctacaccatcggcatggtggagatgggctttaatgatgatgcagcccacggactcttgccggttctttaatcaccctaaacaaatgaccctgcaagacatgggtcggatgtttgggggctggcatctgttccgacacattgaaacccgctttcagctccttgccactaagaatgagggatccttcagccccgtggcgagtcttctctcccagggagagtacctcacgcgtcgggacgatgttaagtacagcagcgatcaccagaaccggtggcgaaaaggcgagcaaccgatgacggggggtattgcttatgcgacggggaaaatgagacccgacgagcaacagtaccctgctatgccccccgaccccccgatcatcacaactaccacaccgcaaggcacgcaagtccgctgcatgaatagcacgcaagcttggtggtcgtgggacacatatatgagctttgcaacactcacagcgctcggtgcacaatggtctttccctccagggcaacgttcagtttctagacgctcgttcaaccaccacaaagcgagaggggccggggaccccaagggacagagatggcacacgcttgttccgctcggcacagagaccatcaccgacagctacatgagtgcgccggcatcagagctggacactaacttctttacgctttacgtagcgcaaggcacaaataaatcgcagcagtacaagttcggcacagctacatacgcgctaaaggaaccggtaatgaagagcgatgcatgggcggtggtacgcgtccagtcagtctggcaactgggtaacaggcaaaggccatacccatgggacgtcaactgggccaacagcaccatgtactgggggtcgcagccctga

SEQ ID NO: 18 - DNA, 651 bp, Chicken anemia virus isolate CAV-10
  gene (1)..(651): VP2 gene of chicken anemia virus isolate CAV-10
atgcacgggaacggcggacaaccggccgctgggggcagtgaatcggcgcttagccgagaggggcaacctgggcccagcggagccgcgcaggggcaagtaatttcaaatgaacgctctccaagaagatactccacccggaccatcaacggtgttcaggccaccaacaagttcacggccgttggaaacccctcactgcagagagatccggattggtatcgctggaattacaatcactctatcgctgtgtggctgcgcgaatgctcgcgctcccacgctaagatctgcaactgcggacaattcagaaagcactggtttcaagaatgtgccggacttgaggaccgatcaacccaagcctccctcgaagaagcgatcctgcgacccctccgagtacagggtaagcgagctaaaagaaagcttgattaccactactcccagccgaccccgaaccgcaagaaggtgtataagactgtaagatggcaagacgagctcgcagaccgagaggcagattttacgccttcagaagaggacggtggcaccacctcaagcgacttcgacgaagatataaatttcgacatcggaggagacagcggtatcgtagacgagcttttaggaaggcctttcacaacccccgccccggtacgtatagtgtga

SEQ ID NO: 19 - DNA, 1482 bp, Fowl adenovirus 4
  gene (1)..(1482): Short fiber gene
ggtcctatccctttttcctatcagggttacgtctactcccccaacgggaacaatgctccgggcccctaaaagaagacattccgaaaacgggaagcccgagaccgaagcgggaccttccccggctccaatcaagcgcgccaaacgcatggtgagagcatcccagcttgacctggtttatcctttcgattacgtggccgaccccgtcggagggctcaacccgccttttttgggaggctcaggacccctagtggaccagggcggacagcttacgctcaacgtcaccgatcccatcatcatcaagaacagatcggtggacttggcccacgaccccagtctcgatgtcaacgcccaaggtcaactggcggtggccgttgaccccgaaggggccctggacatcacccccgatggactggacgtcaaggtcgacccgtccggcggattggattccaccgcgggtggactgggggtcagcgtggacgacaccttgctcgtggatcagggagaactgggcgtacacctcaaccaacaaggacccatcactgccgatagcagtggtatcgacctcgagatcaatcctaacatgttcacggtcaacacctcgaccggaagcggagtgctggaactcaacctaaaagcgcagggaggcatccaagccgacagttcgggagtgggcgtttccgtggatgaaagcctacagattgtcaacaacactctggaagtgaaaccggatcccagcggaccgcttacggtctccgccaatggcctagggctgaagtacgacactaataccctagcggtgaccgcgggcgctttaaccgtggtcggaggggggagcgtctccacacccaatcgctacttttgtctcgggaagtcacagcctcaacacctacaatgccacgccgtcaattccagcgcgaacgccttctcttgcgcctactaccttcaacagtggaacatacaggggctccttgttacctccctctacttgaaattggacagcgccaccatggggaatcgccctggggacctcaactccgccaatgccaaatggttcaccttttgggtgtccgcctatctccagcaatgcaactccgggattcaagcgggaacggtcagcccctccaccgccaccctcacggactttgaacccatggccaataggagcgtgaccagcccatggacgtactcggccaatggatactatgaaccatccatcggggaattccaagtgttcagcccggtggtaacaggtgcctggaacccgggaaacatagggatccgcgtcctccccgtgccggtttcggcctccggagagcgatacacccttctatgctatagtctgcagtgcacgaacgcgagcatttttaatccaaacaacagcggaaccatgatcgtgggacccgtgctctacagctgtccagcggcctccctcccgtaagcgcgccctccccaccgcgtgtcaaataaagagtcatgaacgtt

SEQ ID NO: 20 - DNA, 3510 bp, Infectious bronchitis virus
  gene (1)..(3510): Infectious bronchitis virus strain ArkDPI-derived commercial vaccine D spike glycoprotein gene
atgttggtgaagtcactgtttctagtgaccattttgtttgcactatgtagtgctaatttatatgacaacgaatcttttgtgtattactaccagagtgcttttaggccaggacatggttggcatttatatggaggtgcttatgcagtagttaatgtgtctagtgaaaataataatgcaggtactgccccaagttgcactgctggtgctattggctacagtaagaatctcagtgcggcctcagtagccatgactgcaccactaagtggtatgtcatggtctgccaactctttttgtacagcccactgtaattttacttcttatatagtgtttgttacacattgttataagagcggatctaatagttgtcctttgacaggtcttattccaagcggttatattcgtattgctgctatgaaacatggaagtgctatgcctggtcacttattttataatttaacagtttctgtgactaaatatcctaagtttagatcgctacaatgtgttaataattatacttctgtatatttaaatggtgaccttgttttcacatctaactatactgaagatgttgtagctgcaggtgtccattttaaaagtggtggacctataacttataaagttatgagagaggttaaatccttggcttattttgtcaatggtactgcacatgatgtcattctatgtgatgacacacctagaggtttgttagcatgccaatataatactggcaatttttcagatggcttctatccttttactaatactagtattgttaaggataagtttattgtttatcgtgaaagtagtgtcaatactactttaacattaactaatttcacgtttagtaatgaaagtggtgcccctcctaatacaggtggtgttgacagttttattttataccagacacaaacagctcagagtggttattataattttaacttttcatttctgagtagttttgtttatagggaaagttattatatgtatggatcttaccatccacgttgtagttttagacctgaaacccttaataatggtttgtggtttaattccctttctgtttcattaacatacggtcccattcaaggtggttgtaagcaatctgtatttaatggtaaagcaacttgttgttatgcttattcatacggaggacctcgtggttgtaaaggtgtctatagaggtgagctaacacagcattttgaatgtggtttgttagtttatgttactaagagcgatggctcccgtatacaaactgcaacacaaccacctgtattaacccaaaatttttataataacatcaatttaggtaagtgtgttgattataatatatatggcagaattggccaaggtcttattactaatgtaaccgacttagctgttagttataattatttatcagacgcaggtttggctattttagatacatctggtgccatagacatcttcgttgtacaaggtgaatatggtcctaactattataaggttaatccatgtgaagatgtcaaccaacagtttgtagtttctggtggtaaattagtaggtattctcacttcacgtaatgaaacaggttctcagcttcttgagaaccagttttatattaaaatcactaatggaactcgtcgttctagacgttctgttactgaaaatgttacaaattgcccttatgttagttatggcaagttttgtataaaacctgatggttcaatttctgtaatagtaccaaaagaactggatcagtttgtggcacctttacttaatgttactgaatatgtgctcatacctaacagttttaatttaactgttacagatgagtacatacaaacgcgtatggataagatccaaattaattgcctgcagtatgtttgtggcaattctttggcctgtagaaagctgtttcaacaatatgggcctgtttgtgacaacatattgtctgtagtaaatagtgttggtcaaaaagaagatatggaacttttaaatttctattcttctactaaaccagctcgttttaatacaccagtttttagtaatcttagtactggtgagtttaatatttctcttttgttaacaccccctagtagtcctaggaggcgttcttttattgaagatcttttatttacaagtgttgaatctgtaggattaccaacagatgacgcatacaaaatgtgcactgcaggacctttaggctttcttaaagaccttgcatgtgctcgtgaatataatggtttgcttgtgttgcctcctattataacagcagaaatgcaaactttgtatactagttctttagtagcttctatggcttttggtggtattactgcagctggtgccataccttttgccacacaactgcaggctagaattaatcacttgggtattacccagtcacttttgttgaagaatcaagaaaaaattgctgcttcctttaataaggccattggtcatatgcaggaaggttttaggagtacatctctagcattacaacaaattcaagatgttgttaataagcagagtgctattcttactgagactatggcagcacttaataaaaattttggtgctatttcttctgtgattcaagacatttaccagcaacttgattccatacaagcagatgctcaagtggatcggctcataactggtagattgtcatcactttctgtcttagcatctgctaagcagtcggagtacattagagtgtcacaacagcgtgagttagctactcagaaaattaatgagtgtgttaaatcacagtctattaggtattccttttgtggtaatggacgacatgttttaaccataccacaaaatgcccctaatggtatagtgtttatacactttacttatacaccagagagctttattaatgttactgcaatagtgggtttttgtgtaagtcctgctaatgctagtcagtatgcaatagtgcccgctaatggtaggggtatttttatacaagttaatggtagttactacatcactgcacgagatatgtatatgccaagagatattactgcaggagatatagttacgcttacttcttgtcaagcaaattatgtaagtgtaaataagaccgtcattactacatttgtagacaatgatgattttgattttgctgatgaattgtcaaaatggtggaatgatactaagcatgagctaccagactttgacaaattcaattacacagtacctatacttgacattgatagtgaaattgatcgtattcaaggcgttatacagggtcttaacgactctctaatagaccttgaaacactatcaatactcaaaacttatattaagtggccttggtatgtgtggttagccatagcttttgccactattatcttcatcttaatactaggatggttgtttttcatgactggttgttgtggttgttgttgtggatgctttggcattattcctttaatgagtaagtgtggtaagaaatcttcttattacacgacttttgataatgatgtggtaactgaacaatacagacctaaaaagtctgtttaa

SEQ ID NO: 21 - DNA, 1617 bp, Avian metapneumovirus
  gene (1)..(1617): Gene F of Avian metapneumovirus isolate IT/Ty/A/259-01/03
atggatgtaagaatctgtctcctattgttccttatatctaatcctagtagctgcatacaagaaacatacaatgaagaatcctgcagtactgtaactagaggttataagagtgtgttaaggacagggtggtatacgaatgtatttaacctcgaaatagggaatgttgagaacatcacttgcaatgatggacccagcctaattggcactgagttagtactcacaaagaatgctttgagggagctcaaaacagtgtcagctgatcaagtggctaaggaaagcagactatcctcacccaggagacgtagatttgtactgggtgcaattgcacttggtgttgcgacagctgctgccgtaacagctggtgtagcacttgcaaagacaattagattagagggagaggtgaaggcaattaagaatgccctccggaacacaaatgaggcagtatccacattagggaatggtgtgagggtactagcaactgcagtcaatgacctcaaagaatttataagtaaaaaattgactcctgctattaaccagaacaaatgcaatatagcagatataaagatggcaattagttttggccaaaataacagaaggttcctgaatgtggtgaggcaattctctgatagtgcaggtatcacatcagctgtgtctcttgatttaatgacagatgatgaacttgttagagcaattaacagaatgccaacttcatcaggacagattagtttgatgttgaacaatcgtgccatggttagaaggaaggggtttggtatattgattggtgtttatgatggaacggtcgtttatatggtacaactgcccatattcggcgtgattgagacaccttgttggagggtggtggcagcaccactctgtaggaaaaagaaaggcaattatgcttgtatactgagagaagatcaagggtggtactgtacaaatgctggctctacagcttattatcctaatgaagatgattgtgaggtaagggatgattatgtattttgtgacacagcagctggcattaatgtggccctagaagttgaacagtgcaactataacatatcgacttctaaatacccatgcaaagtcagcacaggtagacaccctgtcagtatggtagccttaacccccctagggggtctagtgtcttgttatgagagtgtaagttgctccataggtagcaataaagtagggataataaaacagctaggcaaagggtgcacccacattcccaacaacgaagctgacacgataaccattgataacactgtgtaccaattgagcaaggttgtaggcgaacagaggaccataaaaggagctccagttgtgaacaattttaacccaatattattccctgaggatcagttcaatgttgcacttgaccaagtatttgagagtatagatagatctcaggacttaatagataagtctaacgacttgctaggtgcagatgccaagagcaaggctggaattgctatagcaatagtagtgctagtcattctaggaatcttctttttacttgcagtgatatattactgttccagagtccggaagaccaaaccaaagcatgattacccggccacgacaggtcatagcagcatggcttatgtcagttaa

SEQ ID NO: 22 - DNA, 25 bp, Synthetic
  misc_feature (1)..(25): Forward primer pCI-Neo
ggctcatgtccaatatgaccgccat

SEQ ID NO: 23 - DNA, 33 bp, Synthetic
  misc_feature (1)..(33): Forward primer EGFP
aaaaaagaattcaccatggtgagcaagggcgag

SEQ ID NO: 24 - DNA, 38 bp, Synthetic
  misc_feature (1)..(38): Reverse primer EGFP
aaaaaagcggccgcttacttgtacagctcgtccatgcc

SEQ ID NO: 25 - DNA, 20 bp, Synthetic
  misc_feature (1)..(20): Forward primer EGFP-I
gagaagcgcgatcacatggt

SEQ ID NO: 26 - DNA, 34 bp, Synthetic
  misc_feature (1)..(34): Forward primer beta-actin
aaaaaaactagttggtcgaggtgagccccacgtt

SEQ ID NO: 27 - DNA, 32 bp, Synthetic
  misc_feature (1)..(32): Reverse primer beta actin
aaaaaagaattcgcccgccgcgcgcttcgctt

SEQ ID NO: 28 - DNA, 44 bp, Synthetic
  misc_feature (1)..(44): Forward primer L2R
aaaaaaactagtcatagtaaatatgggtaacttcttaatagcca

SEQ ID NO: 29 - DNA, 45 bp, Synthetic
  misc_feature (1)..(45): Reverse primer L2R
aaaaaagaattcatggtttgttattggcaaatttaaattaatgtt

SEQ ID NO: 30 - DNA, 34 bp, Synthetic
  misc_feature (1)..(34): Forward primer Luc
aaaaaacctaggttggcaatccggtactgttggt

SEQ ID NO: 31 - DNA, 28 bp, Synthetic
  misc_feature (1)..(28): Reverse primer Luc
aaaaaattcgaagccgccccgactctag

SEQ ID NO: 32 - DNA, 20 bp, Synthetic
  misc_feature (1)..(20): Forward primer SV40
ggcctctgagctattccaga

SEQ ID NO: 33 - DNA, 42 bp, Synthetic
  misc_feature (1)..(42): Forward primer WPRE
aaaaaagcggccgctcaacctctggattacaaaatttgtgaa

SEQ ID NO: 34 - DNA, 33 bp, Synthetic
  misc_feature (1)..(33): Reverse primer WPRE
aaaaaagcggccgcgcccaaagggagatccgac

SEQ ID NO: 35 - DNA, 31 bp, Synthetic
  misc_feature (1)..(31): Forward primer VF1
aaaaaaagatcttacatgaatgacgctgctg

SEQ ID NO: 36 - DNA, 34 bp, Synthetic
  misc_feature (1)..(34): Reverse primer VF1
aaaaaaactagtaaatacaccgagaaataccacg

SEQ ID NO: 37 - DNA, 38 bp, Synthetic
  misc_feature (1)..(38): Forward primer VF2
aaaaaacaattgaaataaagactcagaacgcattttcc

SEQ ID NO: 38 - DNA, 31 bp, Synthetic
  misc_feature (1)..(31): Reverse primer VF2
aaaaaaggtacccccccgcagagaattaaaa

SEQ ID NO: 39 - DNA, 18 bp, Synthetic
  misc_feature (1)..(18): Forward primer E1
acatgaatgacgctgctg

SEQ ID NO: 40 - DNA, 19 bp, Synthetic
  misc_feature (1)..(19): Reverse primer E1
cccccgcagagaattaaaa

SEQ ID NO: 41 - DNA, 496 bp, Avian encephalomyelitis virus
  misc_feature (1)..(496): Internal Ribosomal Entry Site (IRES) from a Canadian isolate of Avian encephalomyelitis virus
tttgaaagaggcctccggggtgtccggaggttctctttcgacccaacccatactggggggtgtgtggggccgtatttggagtgcacggtatatatgcattcccgcatggcaagggcgtgccaccttgccccttgacgcatggtatgtgtcattatttgccttggttaaaccccataaaacgaggcgccacgtgccgaaaatccctttgcgtttcacagaaccatcctaaccatgggtgtagtatgggaatcgtgtatgggggtgattaggatctctcgtagagggataggtgtatcattcaaatccagggagtactctggctctgacattgggacatttgatgtaaccggacctggttcagtatccgggttgtcctgtattgttacggtgtatccgtcttgacacactgaaagggtattcttgggtaatcccttcctactgcctgatagggcggcgtgcccggccacgagagattaagggtagcaatttaaacatg

SEQ ID NO: 42 - DNA, 18 bp, Synthetic
  misc_feature (1)..(18): Forward primer ORF1-2Ver
gcacagtcccaatggctt

SEQ ID NO: 43 - DNA, 20 bp, Synthetic
  misc_feature (1)..(20): Reverse primer ORF1-2Ver
aaattctggtccgttaccga

SEQ ID NO: 44 - DNA, 21 bp, Synthetic
  misc_feature (1)..(21): Forward primer TR2-17-11Ver
gcctactcctcagcctatcac

SEQ ID NO: 45 - DNA, 20 bp, Synthetic
  misc_feature (1)..(20): Reverse primer TR2-17-11Ver
cagtcctctaacgagcacgc

SEQ ID NO: 46 - DNA, 20 bp, Synthetic
  misc_feature (1)..(20): Forward primer CAT
gtgtaggctggagctgcttc

SEQ ID NO: 47 - DNA, 26 bp, Synthetic
  misc_feature (1)..(26): Forward primer ORF1CATSwaI
ggacgtgctttaggtaatttcctccg

SEQ ID NO: 48 - DNA, 25 bp, Synthetic
  misc_feature (1)..(25): Forward primer
ttctttttcccgtttaggtgaggag

SEQ ID NO: 49 - DNA, 28 bp, Synthetic
  misc_feature (1)..(28): Forward primer
atttaaatgtgtaggctggagctgcttc

SEQ ID NO: 50 - DNA, 23 bp, Synthetic
  misc_feature (1)..(23): Reverse primer ORF2CATSwaI
gcgttctgagtctttattggtaa

SEQ ID NO: 51 - DNA, 24 bp, Synthetic
  misc_feature (1)..(24): Reverse primer
actcgaaacacgcgtcacacgcgc

SEQ ID NO: 52 - DNA, 31 bp, Synthetic
  misc_feature (1)..(31): Reverse primer
atttaaatcatatgaatatcctccttagttc

SEQ ID NO: 53 - DNA, 27 bp, Synthetic
  misc_feature (1)..(27): Forward primer TR2-17-11CAT
ccccctggcggccgttggccgccactg

SEQ ID NO: 54 - DNA, 23 bp, Synthetic
  misc_feature (1)..(23): Forward primer
cacccgcgccggacttagtctct

SEQ ID NO: 55 - DNA, 28 bp, Synthetic
  misc_feature (1)..(28): Forward primer
atttaaatgtgtaggctggagctgcttc

SEQ ID NO: 56 - DNA, 27 bp, Synthetic
  misc_feature (1)..(27): Reverse primer TR2-17-11CAT
agtagagattataggaagcggggatta

SEQ ID NO: 57 - DNA, 23 bp, Synthetic
  misc_feature (1)..(23): Reverse primer
tagtggtttttatttaaacgaga

SEQ ID NO: 58 - DNA, 31 bp, Synthetic; identical to SEQ ID NO: 52
  misc_feature (1)..(31): Reverse primer

SEQ ID NO: 59 - DNA, 25 bp, Synthetic
  misc_feature (1)..(25): Forward primer ORF17CATSwaI
tccccctggcggccgagggccgcca

SEQ ID NO: 60 - DNA, 26 bp, Synthetic
  misc_feature (1)..(26): Forward primer
ctgcacccgcgccggacttagtctct

SEQ ID NO: 61 - DNA, 28 bp, Synthetic
  misc_feature (1)..(28): Forward primer
atttaaatgtgtaggctggagctgcttc

SEQ ID NO: 62 - DNA, 26 bp, Synthetic
  misc_feature (1)..(26): Reverse primer ORF17CATSwaI
gatacgaagaaggataggagcagaat

SEQ ID NO: 63 - DNA, 22 bp, Synthetic
  misc_feature (1)..(22): Reverse primer
cgaggatacggtagttgactcc

SEQ ID NO: 64 - DNA, 33 bp, Synthetic
  misc_feature (1)..(33): Reverse primer
atatttaaatcatatgaatatcctccttagttc

SEQ ID NO: 65 - DNA, 34 bp, Synthetic
  misc_feature (1)..(34): Forward primer EGFPcaSwaI
agctgcatttaaatgtattaccgccatgcattag

SEQ ID NO: 66 - DNA, 33 bp, Synthetic
  misc_feature (1)..(33): Reverse primer EGFPcaSwaI
agctgcatttaaatccacaactagaatgcagtg

SEQ ID NO: 67 - DNA, 36 bp, Synthetic
  misc_feature (1)..(36): Forward primer mCherry
agctgcatttaaatatggtgagcaagggcgaggagg

SEQ ID NO: 68 - DNA, 39 bp, Synthetic
  misc_feature (1)..(39): Reverse primer mCherry
agctgcatttaaatctacttgtacagctcgtccatgccg